European Patent Specification EP 3 924 048 B1, published June 10, 2026. Title: Methods of reactivating proliferative capacity in non-proliferative tissues. Applicant: Cambridge Enterprise Limited. The sequence listing filed with the application follows.

SEQUENCE LISTING (38 sequences)

SEQ ID NO: 1 - protein, 753 aa, Artificial Sequence
  MycERT2
MPLNVSFTNRNYDLDYDSVQPYFYCDEEENFYQQQQQSELQPPAPSEDIWKKFELLPTPPLSPSRRSGLCSPSYVAVTPFSLRGDNDGGGGSFSTADQLEMVTELLGGDMVNQSFICDPDDETFIKNIIIQDCMWSGFSAAAKLVSEKLASYQAARKDSGSPNPARGHSVCSTSSLYLQDLSAAASECIDPSVVFPYPLNDSSSPKSCASQDSSAFSPSSDSLLSSTESSPQGSPEPLVLHEETPPTTSSDSEEEQEDEEEIDVVSVEKRQAPGKRSESGSPSAGGHSKPPHSPLVLKRCHVSTHQHNYAAPPSTRKDYPAAKRVKLDSVRVLRQISNNRKCTSPRSSDTEENVKRRTHNVLERQRRNELKRSFFALRDQIPELENNEKAPKVVILKKATAYILSVQAEEQKLISEEDLLRKRREQLKHKLEQLRDPGSAGDMRAANLWPSPLMIKRSKKNSLALSLTADQMVSALLDAEPPILYSEYDPTRPFSEASMMGLLTNLADRELVHMINWAKRVPGFVDLTLHDQVHLLECAWLEILMIGLVWRSMEHPVKLLFAPNLLLDRNQGKCVEGMVEIFDMLLATSSRFRMMNLQGEEFVCLKSIILLNSGVYTFLSSTLKSLEEKDHIHRVLDKITDTLIHLMAKAGLTLQQQHQRLAQLLLILSHIRHMSNKGMEHLYSMKCKNVVPLYDLLLEAADAHRLHAPTSRGGASVEETDQSHLATAGSTSSHSLQKYYITGEAEGFPATVQ

SEQ ID NO: 2 - DNA, 2264 bp, Artificial Sequence
  MycERT2
atgcccctcaacgttagcttcaccaacaggaactatgacctcgactacgactcggtgcagccgtatttctactgcgacgaggaggagaacttctaccagcagcagcagcagagcgagctgcagcccccggcgcccagcgaggatatctggaagaaattcgagctgctgcccaccccgcccctgtcccctagccgccgctccgggctctgctcgccctcctacgttgcggtcacacccttctcccttcggggagacaacgacggcggtggcgggagcttctccacggccgaccagctggagatggtgaccgagctgctgggaggagacatggtgaaccagagtttcatctgcgacccggacgacgagaccttcatcaaaaacatcatcatccaggactgtatgtggagcggcttctcggccgccgccaagctcgtctcagagaagctggcctcctaccaggctgcgcgcaaagacagcggcagcccgaaccccgcccgcggccacagcgtctgctccacctccagcttgtacctgcaggatctgagcgccgccgcctcagagtgcatcgacccctcggtggtcttcccctaccctctcaacgacagcagctcgcccaagtcctgcgcctcgcaagactccagcgccttctctccgtcctcggattctctgctctcctcgacggagtcctccccgcagggcagccccgagcccctggtgctccatgaggagacaccgcccaccaccagcagcgactctgaggaggaacaagaagatgaggaagaaatcgatgttgtttctgtggaaaagaggcaggctcctggcaaaaggtcagagtctggatcaccttctgctggaggccacagcaaacctcctcacagcccactggtcctcaagaggtgccacgtctccacacatcagcacaactacgcagcgcctccctccactcggaaggactatcctgctgccaagagggtcaagttggacagtgtcagagtcctgagacagatcagcaacaaccgaaaatgcaccagccccaggtcctcggacaccgaggagaatgtcaagaggcgaacacacaacgtcttggagcgccagaggaggaacgagctaaaacggagcttttttgccctgcgtgaccagatcccggagttggaaaacaatgaaaaggcccccaaggtagttatccttaaaaaagccacagcatacatcctgtccgtccaagcagaggagcaaaagctcatttctgaagaggacttgttgcggaaacgacgagaacagttgaaacacaaacttgaacagctacgggatccggggtctgctggagacatgagagctgccaacctttggccaagcccgctcatgatcaaacgctctaagaagaacagcctggccttgtccctgacggccgaccagatggtcagtgccttgttggatgctgagccccccatactctattccgagtatgatcctaccagacccttcagtgaagcttcgatgatgggcttactgaccaacctggcagacagggagctggttcacatgatcaactgggcgaagagggtgccaggctttgtggatttgaccctccatgatcaggtccaccttctagaatgtgcctggctagagatcctgatgattggtctcgtctggcgctccatggagcacccagtgaagctactgtttgctcctaacttgctcttggacaggaaccagggaaaatgtgtagagggcatggtggagatcttcgacatgctgctggctacatcatctcggttccgcatgatgaatctgcagggagaggagtttgtgtgcctcaaatctattattttgcttaattctggagtgtacacatttctgtccagcaccctgaagtctctggaagagaaggaccatatccaccgagtcctggacaagatcacagacactttgatccacctgatggccaaggcaggcctgaccctgcagcagcagcaccagcggctggcccagctcctcctcatcctctcccacatcaggcacatgagtaacaaaggcatggagcatctgtacagcatgaagtgcaagaacgtggtgcccctctatgacctgctgctggaggcggcggacgcccaccgcctacatgcgcccactagccgtggaggggcatccgtggaggagacggaccaaagccacttggccactgcgggctctacttcatcgcattccttgcaaaagtattacatcacgggggaggcagagggtttccctgccacagtctgacaatt

SEQ ID NO: 3 - DNA, 2590 bp, Artificial Sequence
  CAG promoter
cggccgcccaccctccccttcctctgggggagtcgttttacccgccgccggccgggcctcgtcgtctgattggctctcggggcccagaaaactggcccttgccattggctcgtgttcgtgcaagttgagtccatccgccggccagcgggggcggcgaggaggcgctcccaggttccggccctcccctcggccccgcgccgcagagtctggccgcgcgcccctgcgcaacgtggcaggaagcgcgcgctgggggcggggacgggcagtagggctgagcggctgcggggcgggtgcaagcacgtttccgacttgagttgcctcaagaggggcgtgctgagccagacctccatcgcgcactccggggagtggagggaaggagcgagggctcagttgggctgttttggaggcaggaagcacttgctctcccaaagtcgctctgagttgttatcagtaagggagctgcagtggagtaggcggggagaaggccgcacccttctccggaggggggaggggagtgttgcaatacctttctgggagttctctgctgcctcctggcttctgaggaccgccctgggcctgggagaatcccttccccctcttccctcgtgatctgcaactccagtctttctaggtaaccgatatccctgcaggttttcgacattgattattgactagttattaatagtaatcaattacggggtcattagttcatagcccatatatggagttccgcgttacataacttacggtaaatggcccgcctggctgaccgcccaacgacccccgcccattgacgtcaataatgacgtatgttcccatagtaacgccaatagggactttccattgacgtcaatgggtggagtatttacggtaaactgcccacttggcagtacatcaagtgtatcatatgccaagtacgccccctattgacgtcaatgacggtaaatggcccgcctggcattatgcccagtacatgaccttatgggactttcctacttggcagtacatctacgtattagtcatcgctattaccatggtcgaggtgagccccacgttctgcttcactctccccatctcccccccctccccacccccaattttgtatttatttattttttaattattttgtgcagcgatgggggcggggggggggggggcgcgcgccaggcggggcggggcggggcgaggggcggggcggggcgaggcggagaggtgcggcggcagccaatcagagcggcgcgctccgaaagtttccttttatggcgaggcggcggcggcggcggccctataaaaagcgaagcgcgcggcgggcgggagtcgctgcgttgccttcgccccgtgccccgctccgcgccgcctcgcgccgcccgccccggctctgactgaccgcgttactcccacaggtgagcgggcgggacggcccttctcctccgggctgtaattagcgcttggtttaatgacggctcgtttcttttctgtggctgcgtgaaagccttaaagggctccgggagggccctttgtgcgggggggagcggctcggggggtgcgtgcgtgtgtgtgtgcgtggggagcgccgcgtgcggcccgcgctgcccggcggctgtgagcgctgcgggcgcggcgcggggctttgtgcgctccgcgtgtgcgcgaggggagcgcggccgggggcggtgccccgcggtgcgggggggctgcgaggggaacaaaggctgcgtgcggggtgtgtgcgtgggggggtgagcagggggtgtgggcgcggcggtcgggctgtaacccccccctgcacccccctccccgagttgctgagcacggcccggcttcgggtgcggggctccgtgcggggcgtggcgcggggctcgccgtgccgggcggggggtggcggcaggtgggggtgccgggcggggcggggccgcctcgggccggggagggctcgggggaggggcgcggcggccccggagcgccggcggctgtcgaggcgcggcgagccgcagccattgccttttatggtaatcgtgcgagagggcgcagggacttcctttgtcccaaatctggcggagccgaaatctgggaggcgccgccgcaccccctctagcgggcgcgggcgaagcggtgcggcgccggcaggaaggaaatgggcggggagggccttcgtgcgtcgccgcgccgccgtccccttctccatctccagcctcggggctgccgcagggggacggctgccttcgggggggacggggcagggcggggttcggcttctggcgtgtgaccggcggctctagaagcgttggggtgagtactccctctcaaaagcgggcatgacttctgcgctaagattgtcagtttccaaaaacgaggaggatttgatattcacctggcccgcggtgatgcctttgagggtggccgcgtccatctggtcagaaaagacaatctttttgttgtcaagcttgaggtgtggcaggcttgagatctggccatacacttgagtgacattgacatccactttgcctttctctccacaggtgtccactcccagggcggcctccggagcgatcgccggtccgcctaggctagccggccgcgtcgacttaat

SEQ ID NO: 4 - DNA, 429 bp, Artificial Sequence
  Troponin T promoter
tctctcggggtgggggataaaagcagtctgggctttcacatgacagcatctggggctgcggcagagggtcgggtccgaagcgctgccttatcagcgtccccagccctgggaggtgacagctggctggcttgtgtcagcccctcgggcactcacgtatctccatccgacgggtttaaaatagcaaaactctgaggccacacaatagcttgggcttatatgggctcctgtgggggaagggggagcacggagggggccggggccgctgctgccaaaatagcagctcacaagtgttgcattcctctctgggcgccgggcacattcctgctggctctgcccgccccggggtgggcgccggggggaccttaaagcctctgccccccaaggagcccttcccagacagccgccggcacccaccgctccgtgggacct

SEQ ID NO: 5 - protein, 726 aa, Artificial Sequence
  Cyclin T1 amino acid sequence
MEGERKNNNKRWYFTREQLENSPSRRFGVDPDKELSYRQQAANLLQDMGQRLNVSQLTINTAIVYMHRFYMIQSFTQFPGNSVAPAALFLAAKVEEQPKKLEHVIKVAHTCLHPQESLPDTRSEAYLQQVQDLVILESIILQTLGFELTIDHPHTHVVKCTQLVRASKDLAQTSYFMATNSLHLTTFSLQYTPPVVACVCIHLACKWSNWEIPVSTDGKHWWEYVDATVTLELLDELTHEFLQILEKTPNRLKRIWNWRACEAAKKTKADDRGTDEKTSEQTILNMISQSSSDTTIAGLMSMSTSTTSAVPSLPVSEESSSNLTSVEMLPGKRWLSSQPSFKLEPTQGHRTSENLALTGVDHSLPQDGSNAFISQKQNSKSVPSAKVSLKEYRAKHAEELAAQKRQLENMEANVKSQYAYAAQNLLSHHDSHSSVILKMPIEGSENPERPFLEKADKTALKMRIPVAGGDKAASSKPEEIKMRIKVHAAADKHNSVEDSVTKSREHKEKHKTHPSNHHHHHNHHSHKHSHSQLPVGTGNKRPGDPKHSSQTSNLAHKTYSLSSSFSSSSSTRKRGPSEETGGAVFDHPAKIAKSTKSSSLNFSFPSLPTMGQMPGHSSDTSGLSFSQPSCKTRVPHSKLDKGPTGANGHNTTQTIDYQDTVNMLHSLLSAQGVQPTQPTAFEFVRPYSDYLNPRSGGISSRSGNTDKPRPPPLPSEPPPPLPPLPK

SEQ ID NO: 6 - DNA, 2181 bp, Artificial Sequence
  Cyclin T1 nucleic acid sequence
atggagggagagaggaagaacaacaacaaacggtggtatttcactcgagaacagctggaaaatagcccatcccgtcgttttggcgtggacccagataaagaactttcttatcgccagcaggcggccaatctgcttcaggacatggggcagcgtcttaacgtctcacaattgactatcaacactgctatagtatacatgcatcgattctacatgattcagtccttcacacagttccctggaaattctgtggctccagcagccttgtttctagcagctaaagtggaggagcagcccaaaaaattggaacatgtcatcaaggtagcacatacttgtctccatcctcaggaatcccttcctgatactagaagtgaggcttatttgcaacaagttcaagatctggtcattttagaaagcataattttgcagactttaggctttgaactaacaattgatcacccacatactcatgtagtaaagtgcactcaacttgttcgagcaagcaaggacttagcacagacttcttacttcatggcaaccaacagcctgcatttgaccacatttagcctgcagtacacacctcctgtggtggcctgtgtctgcattcacctggcttgcaagtggtccaattgggagatcccagtctcaactgacgggaagcactggtgggagtatgttgacgccactgtgaccttggaacttttagatgaactgacacatgagtttctacagattttggagaaaactcccaacaggctcaaacgcatttggaattggagggcatgcgaggctgccaagaaaacaaaagcagatgaccgaggaacagatgaaaagacttcagagcagacaatcctcaatatgatttcccagagctcttcagacacaaccattgcaggtttaatgagcatgtcaacttctaccacaagtgcagtgccttccctgccagtctccgaagagtcatccagcaacttaaccagtgtggagatgttgccgggcaagcgttggctgtcctcccaaccttctttcaaactagaacctactcagggtcatcggactagtgagaatttagcacttacaggagttgatcattccttaccacaggatggttcaaatgcatttatttcccagaagcagaatagtaagagtgtgccatcagctaaagtgtcactgaaagaataccgcgcgaagcatgcagaagaattggctgcccagaagaggcaactggagaacatggaagccaatgtgaagtcacaatatgcatatgctgcccagaatctcctttctcatcatgatagccattcttcagtcattctaaaaatgcccatagagggttcagaaaaccccgagcggccttttctggaaaaggctgacaaaacagctctcaaaatgagaatcccagtggcaggtggagataaagctgcgtcttcaaaaccagaggagataaaaatgcgcataaaagtccatgctgcagctgataagcacaattctgtagaggacagtgttacaaagagccgagagcacaaagaaaagcacaagactcacccatctaatcatcatcatcatcataatcaccactcacacaagcactctcattcccaacttccagttggtactgggaacaaacgtcctggtgatccaaaacatagtagccagacaagcaacttagcacataaaacctatagcttgtctagttctttttcctcttccagttctactcgtaaaaggggaccctctgaagagactggaggggctgtgtttgatcatccagccaagattgccaagagtactaaatcctcttccctaaatttctccttcccttcacttcctacaatgggtcagatgcctgggcatagctcagacacaagtggcctttccttttcacagcccagctgtaaaactcgtgtccctcattcgaaactggataaagggcccactggggccaatggtcacaacacgacccagacaatagactatcaagacactgtgaatatgcttcactccctgctcagtgcccagggtgttcagcccactcagcccactgcatttgaatttgttcgtccttatagtgactatctgaatcctcggtctggtggaatctcctcgagatctggcaatacagacaaaccccggccaccacctctgccatcagaacctcctccaccacttccaccccttcctaagtaa

SEQ ID NO: 7 - protein, 372 aa, Artificial Sequence
  CDK9 amino acid sequence
MAKQYDSVECPFCDEVSKYEKLAKIGQGTFGEVFKARHRKTGQKVALKKVLMENEKEGFPITALREIKILQLLKHENVVNLIEICRTKASPYNRCKGSIYLVFDFCEHDLAGLLSNVLVKFTLSEIKRVMQMLLNGLYYIHRNKILHRDMKAANVLITRDGVLKLADFGLARAFSLAKNSQPNRYTNRVVTLWYRPPELLLGERDYGPPIDLWGAGCIMAEMWTRSPIMQGNTEQHQLALISQLCGSITPEVWPNVDNYELYEKLELVKGQKRKVKDRLKAYVRDPYALDLIDKLLVLDPAQRIDSDDALNHDFFWSDPMPSDLKGMLSTHLTSMFEYLAPPRRKGSQITQQSTNQSRNPATTNQTEFERVF

SEQ ID NO: 8 - DNA, 1119 bp, Artificial Sequence
  CDK9 nucleic acid sequence
atggcaaagcagtacgactcggtggagtgccctttttgtgatgaagtttccaaatacgagaagctcgccaagatcggccaaggcaccttcggggaggtgttcaaggccaggcaccgcaagaccggccagaaggtggctctgaagaaggtgctgatggaaaacgagaaggaggggttccccattacagccttgcgggagatcaagatccttcagcttctaaaacacgagaatgtggtcaacttgattgagatttgtcgaaccaaagcttccccctataaccgctgcaagggtagtatatacctggtgttcgacttctgcgagcatgaccttgctgggctgttgagcaatgttttggtcaagttcacgctgtctgagatcaagagggtgatgcagatgctgcttaacggcctctactacatccacagaaacaagatcctgcatagggacatgaaggctgctaatgtgcttatcactcgtgatggggtcctgaagctggcagactttgggctggcccgggccttcagcctggccaagaacagccagcccaaccgctacaccaaccgtgtggtgacactctggtaccggcccccggagctgttgctcggggagcgggactacggcccccccattgacctgtggggtgctgggtgcatcatggcagagatgtggacccgcagccccatcatgcagggcaacacggagcagcaccaactcgccctcatcagtcagctctgcggctccatcacccctgaggtgtggccaaacgtggacaactatgagctgtacgaaaagctggagctggtcaagggccagaagcggaaggtgaaggacaggctgaaggcctatgtgcgtgacccatacgcactggacctcatcgacaagctgctggtgctggaccctgcccagcgcatcgacagcgatgacgccctcaaccacgacttcttctggtccgaccccatgccctccgacctcaagggcatgctctccacccacctgacgtccatgttcgagtacttggcaccaccgcgccggaagggcagccagatcacccagcagtccaccaaccagagtcgcaatcccgccaccaccaaccagacggagtttgagcgcgtcttctga

SEQ ID NO: 9 - DNA, 2291 bp, Artificial Sequence
  MycERTM
atgcccctcaacgttagcttcaccaacaggaactatgacctcgactacgactcggtgcagccgtatttctactgcgacgaggaggagaacttctaccagcagcagcagcagagcgagctgcagcccccggcgcccagcgaggatatctggaagaaattcgagctgctgcccaccccgcccctgtcccctagccgccgctccgggctctgctcgccctcctacgttgcggtcacacccttctcccttcggggagacaacgacggcggtggcgggagcttctccacggccgaccagctggagatggtgaccgagctgctgggaggagacatggtgaaccagagtttcatctgcgacccggacgacgagaccttcatcaaaaacatcatcatccaggactgtatgtggagcggcttctcggccgccgccaagctcgtctcagagaagctggcctcctaccaggctgcgcgcaaagacagcggcagcccgaaccccgcccgcggccacagcgtctgctccacctccagcttgtacctgcaggatctgagcgccgccgcctcagagtgcatcgacccctcggtggtcttcccctaccctctcaacgacagcagctcgcccaagtcctgcgcctcgcaagactccagcgccttctctccgtcctcggattctctgctctcctcgacggagtcctccccgcagggcagccccgagcccctggtgctccatgaggagacaccgcccaccaccagcagcgactctgaggaggaacaagaagatgaggaagaaatcgatgttgtttctgtggaaaagaggcaggctcctggcaaaaggtcagagtctggatcaccttctgctggaggccacagcaaacctcctcacagcccactggtcctcaagaggtgccacgtctccacacatcagcacaactacgcagcgcctccctccactcggaaggactatcctgctgccaagagggtcaagttggacagtgtcagagtcctgagacagatcagcaacaaccgaaaatgcaccagccccaggtcctcggacaccgaggagaatgtcaagaggcgaacacacaacgtcttggagcgccagaggaggaacgagctaaaacggagcttttttgccctgcgtgaccagatcccggagttggaaaacaatgaaaaggcccccaaggtagttatccttaaaaaagccacagcatacatcctgtccgtccaagcagaggagcaaaagctcatttctgaagaggacttgttgcggaaacgacgagaacagttgaaacacaaacttgaacagctacgggatccacgaaatgaaatgggtgcttcaggagacatgagggctgccaacctttggccaagccctcttgtgattaagcacactaagaagaatagccctgccttgtccttgacagctgaccagatggtcagtgccttgttggatgctgaaccgcccatgatctattctgaatatgatccttctagacccttcagtgaagcctcaatgatgggcttattgaccaacctagcagatagggagctggttcatatgatcaactgggcaaagagagtgccaggctttggggacttgaatctccatgatcaggtccaccttctcgagtgtgcctggctggagattctgatgattggtctcgtctggcgctccatggaacacccggggaagctcctgtttgctcctaacttgctcctggacaggaatcaaggtaaatgtgtggaaggcatggtggagatctttgacatgttgcttgctacgtcaagtcggttccgcatgatgaacctgcagggtgaagagtttgtgtgcctcaaatccatcattttgcttaattccggagtgtacacgtttctgtccagcaccttgaagtctctggaagagaaggaccacatccaccgtgtcctggacaagatcacagacactttgatccacctgatggccaaagctggcctgactctgcagcagcagcatcgccgcctagctcagctccttctcattctttcccatatccggcacatgagtaacaaacgcatggagcatctctacaacatgaaatgcaagaacgtggtacccctctatgacctgctcctggagatgttggatgcccaccgccttcatgccccagccagtcgcatgggagtgcccccagaggagcccagccagacccagctggccaccaccagctccacttcagcacattccttacaaacctactacatacccccggaagcagagggcttccccaacacgatctgagagctcctactagtgaattc

SEQ ID NO: 10 - protein, 762 aa, Artificial Sequence
  MycERTM
MPLNVSFTNRNYDLDYDSVQPYFYCDEEENFYQQQQQSELQPPAPSEDIWKKFELLPTPPLSPSRRSGLCSPSYVAVTPFSLRGDNDGGGGSFSTADQLEMVTELLGGDMVNQSFICDPDDETFIKNIIIQDCMWSGFSAAAKLVSEKLASYQAARKDSGSPNPARGHSVCSTSSLYLQDLSAAASECIDPSVVFPYPLNDSSSPKSCASQDSSAFSPSSDSLLSSTESSPQGSPEPLVLHEETPPTTSSDSEEEQEDEEEIDVVSVEKRQAPGKRSESGSPSAGGHSKPPHSPLVLKRCHVSTHQHNYAAPPSTRKDYPAAKRVKLDSVRVLRQISNNRKCTSPRSSDTEENVKRRTHNVLERQRRNELKRSFFALRDQIPELENNEKAPKVVILKKATAYILSVQAEEQKLISEEDLLRKRREQLKHKLEQLRDPRNEMGASGDMRAANLWPSPLVIKHTKKNSPALSLTADQMVSALLDAEPPMIYSEYDPSRPFSEASMMGLLTNLADRELVHMINWAKRVPGFGDLNLHDQVHLLECAWLEILMIGLVWRSMEHPGKLLFAPNLLLDRNQGKCVEGMVEIFDMLLATSSRFRMMNLQGEEFVCLKSIILLNSGVYTFLSSTLKSLEEKDHIHRVLDKITDTLIHLMAKAGLTLQQQHRRLAQLLLILSHIRHMSNKRMEHLYNMKCKNVVPLYDLLLEMLDAHRLHAPASRMGVPPEEPSQTQLATTSSTSAHSLQTYYIPPEAEGFPNTIELLLVN

SEQ ID NO: 11 - protein, 454 aa, Artificial Sequence
  c-myc
MDFFRVVENQQPPATMPLNVSFTNRNYDLDYDSVQPYFYCDEEENFYQQQQQSELQPPAPSEDIWKKFELLPTPPLSPSRRSGLCSPSYVAVTPFSLRGDNDGGGGSFSTADQLEMVTELLGGDMVNQSFICDPDDETFIKNIIIQDCMWSGFSAAAKLVSEKLASYQAARKDSGSPNPARGHSVCSTSSLYLQDLSAAASECIDPSVVFPYPLNDSSSPKSCASQDSSAFSPSSDSLLSSTESSPQGSPEPLVLHEETPPTTSSDSEEEQEDEEEIDVVSVEKRQAPGKRSESGSPSAGGHSKPPHSPLVLKRCHVSTHQHNYAAPPSTRKDYPAAKRVKLDSVRVLRQISNNRKCTSPRSSDTEENVKRRTHNVLERQRRNELKRSFFALRDQIPELENNEKAPKVVILKKATAYILSVQAEEQKLISEEDLLRKRREQLKHKLEQLRNSCA

SEQ ID NO: 12 - DNA, 1365 bp, Artificial Sequence
  c-myc
ctggatttttttcgggtagtggaaaaccagcagcctcccgcgacgatgcccctcaacgttagcttcaccaacaggaactatgacctcgactacgactcggtgcagccgtatttctactgcgacgaggaggagaacttctaccagcagcagcagcagagcgagctgcagcccccggcgcccagcgaggatatctggaagaaattcgagctgctgcccaccccgcccctgtcccctagccgccgctccgggctctgctcgccctcctacgttgcggtcacacccttctcccttcggggagacaacgacggcggtggcgggagcttctccacggccgaccagctggagatggtgaccgagctgctgggaggagacatggtgaaccagagtttcatctgcgacccggacgacgagaccttcatcaaaaacatcatcatccaggactgtatgtggagcggcttctcggccgccgccaagctcgtctcagagaagctggcctcctaccaggctgcgcgcaaagacagcggcagcccgaaccccgcccgcggccacagcgtctgctccacctccagcttgtacctgcaggatctgagcgccgccgcctcagagtgcatcgacccctcggtggtcttcccctaccctctcaacgacagcagctcgcccaagtcctgcgcctcgcaagactccagcgccttctctccgtcctcggattctctgctctcctcgacggagtcctccccgcagggcagccccgagcccctggtgctccatgaggagacaccgcccaccaccagcagcgactctgaggaggaacaagaagatgaggaagaaatcgatgttgtttctgtggaaaagaggcaggctcctggcaaaaggtcagagtctggatcaccttctgctggaggccacagcaaacctcctcacagcccactggtcctcaagaggtgccacgtctccacacatcagcacaactacgcagcgcctccctccactcggaaggactatcctgctgccaagagggtcaagttggacagtgtcagagtcctgagacagatcagcaacaaccgaaaatgcaccagccccaggtcctcggacaccgaggagaatgtcaagaggcgaacacacaacgtcttggagcgccagaggaggaacgagctaaaacggagcttttttgccctgcgtgaccagatcccggagttggaaaacaatgaaaaggcccccaaggtagttatccttaaaaaagccacagcatacatcctgtccgtccaagcagaggagcaaaagctcatttctgaagaggacttgttgcggaaacgacgagaacagttgaaacacaaacttgaacagctacggaactcttgtgcgtaa

SEQ ID NO: 13 - RNA, 2181 nt, Artificial Sequence
  Cyclin T1
auggagggagagaggaagaacaacaacaaacggugguauuucacucgagaacagcuggaaaauagcccaucccgucguuuuggcguggacccagauaaagaacuuucuuaucgccagcaggcggccaaucugcuucaggacauggggcagcgucuuaacgucucacaauugacuaucaacacugcuauaguauacaugcaucgauucuacaugauucaguccuucacacaguucccuggaaauucuguggcuccagcagccuuguuucuagcagcuaaaguggaggagcagcccaaaaaauuggaacaugucaucaagguagcacauacuugucuccauccucaggaaucccuuccugauacuagaagugaggcuuauuugcaacaaguucaagaucuggucauuuuagaaagcauaauuuugcagacuuuaggcuuugaacuaacaauugaucacccacauacucauguaguaaagugcacucaacuuguucgagcaagcaaggacuuagcacagacuucuuacuucauggcaaccaacagccugcauuugaccacauuuagccugcaguacacaccuccugugguggccugugucugcauucaccuggcuugcaagugguccaauugggagaucccagucucaacugacgggaagcacuggugggaguauguugacgccacugugaccuuggaacuuuuagaugaacugacacaugaguuucuacagauuuuggagaaaacucccaacaggcucaaacgcauuuggaauuggagggcaugcgaggcugccaagaaaacaaaagcagaugaccgaggaacagaugaaaagacuucagagcagacaauccucaauaugauuucccagagcucuucagacacaaccauugcagguuuaaugagcaugucaacuucuaccacaagugcagugccuucccugccagucuccgaagagucauccagcaacuuaaccaguguggagauguugccgggcaagcguuggcuguccucccaaccuucuuucaaacuagaaccuacucagggucaucggacuagugagaauuuagcacuuacaggaguugaucauuccuuaccacaggaugguucaaaugcauuuauuucccagaagcagaauaguaagagugugccaucagcuaaagugucacugaaagaauaccgcgcgaagcaugcagaagaauuggcugcccagaagaggcaacuggagaacauggaagccaaugugaagucacaauaugcauaugcugcccagaaucuccuuucucaucaugauagccauucuucagucauucuaaaaaugcccauagaggguucagaaaaccccgagcggccuuuucuggaaaaggcugacaaaacagcucucaaaaugagaaucccaguggcagguggagauaaagcugcgucuucaaaaccagaggagauaaaaaugcgcauaaaaguccaugcugcagcugauaagcacaauucuguagaggacaguguuacaaagagccgagagcacaaagaaaagcacaagacucacccaucuaaucaucaucaucaucauaaucaccacucacacaagcacucucauucccaacuuccaguugguacugggaacaaacguccuggugauccaaaacauaguagccagacaagcaacuuagcacauaaaaccuauagcuugucuaguucuuuuuccucuuccaguucuacucguaaaaggggacccucugaagagacuggaggggcuguguuugaucauccagccaagauugccaagaguacuaaauccucuucccuaaauuucuccuucccuucacuuccuacaaugggucagaugccugggcauagcucagacacaaguggccuuuccuuuucacagcccagcuguaaaacucgugucccucauucgaaacuggauaaagggcccacuggggccaauggucacaacacgacccagacaauagacuaucaagacacugugaauaugcuucacucccugcucagugcccaggguguucagcccacucagcccacugcauuugaauuuguucguccuuauagugacuaucugaauccucggucugguggaaucuccucgagaucuggcaauacagacaaaccccggccaccaccucugccaucagaaccuccuccaccacuuccaccccuuccuaaguaa

SEQ ID NO: 14 - RNA, 1119 nt, Artificial Sequence
  CDK9
auggcaaagcaguacgacucgguggagugcccuuuuugugaugaaguuuccaaauacgagaagcucgccaagaucggccaaggcaccuucggggagguguucaaggccaggcaccgcaagaccggccagaagguggcucugaagaaggugcugauggaaaacgagaaggagggguuccccauuacagccuugcgggagaucaagauccuucagcuucuaaaacacgagaauguggucaacuugauugagauuugucgaaccaaagcuucccccuauaaccgcugcaaggguaguauauaccugguguucgacuucugcgagcaugaccuugcugggcuguugagcaauguuuuggucaaguucacgcugucugagaucaagagggugaugcagaugcugcuuaacggccucuacuacauccacagaaacaagauccugcauagggacaugaaggcugcuaaugugcuuaucacucgugaugggguccugaagcuggcagacuuugggcuggcccgggccuucagccuggccaagaacagccagcccaaccgcuacaccaaccguguggugacacucugguaccggcccccggagcuguugcucggggagcgggacuacggcccccccauugaccuguggggugcugggugcaucauggcagagauguggacccgcagccccaucaugcagggcaacacggagcagcaccaacucgcccucaucagucagcucugcggcuccaucaccccugagguguggccaaacguggacaacuaugagcuguacgaaaagcuggagcuggucaagggccagaagcggaaggugaaggacaggcugaaggccuaugugcgugacccauacgcacuggaccucaucgacaagcugcuggugcuggacccugcccagcgcaucgacagcgaugacgcccucaaccacgacuucuucugguccgaccccaugcccuccgaccucaagggcaugcucuccacccaccugacguccauguucgaguacuuggcaccaccgcgccggaagggcagccagaucacccagcaguccaccaaccagagucgcaaucccgccaccaccaaccagacggaguuugagcgcgucuucuga

SEQ ID NO: 15 - RNA, 1365 nt, Artificial Sequence
  c-myc
cuggauuuuuuucggguaguggaaaaccagcagccucccgcgacgaugccccucaacguuagcuucaccaacaggaacuaugaccucgacuacgacucggugcagccguauuucuacugcgacgaggaggagaacuucuaccagcagcagcagcagagcgagcugcagcccccggcgcccagcgaggauaucuggaagaaauucgagcugcugcccaccccgccccuguccccuagccgccgcuccgggcucugcucgcccuccuacguugcggucacacccuucucccuucggggagacaacgacggcgguggcgggagcuucuccacggccgaccagcuggagauggugaccgagcugcugggaggagacauggugaaccagaguuucaucugcgacccggacgacgagaccuucaucaaaaacaucaucauccaggacuguauguggagcggcuucucggccgccgccaagcucgucucagagaagcuggccuccuaccaggcugcgcgcaaagacagcggcagcccgaaccccgcccgcggccacagcgucugcuccaccuccagcuuguaccugcaggaucugagcgccgccgccucagagugcaucgaccccucgguggucuuccccuacccucucaacgacagcagcucgcccaaguccugcgccucgcaagacuccagcgccuucucuccguccucggauucucugcucuccucgacggaguccuccccgcagggcagccccgagccccuggugcuccaugaggagacaccgcccaccaccagcagcgacucugaggaggaacaagaagaugaggaagaaaucgauguuguuucuguggaaaagaggcaggcuccuggcaaaaggucagagucuggaucaccuucugcuggaggccacagcaaaccuccucacagcccacugguccucaagaggugccacgucuccacacaucagcacaacuacgcagcgccucccuccacucggaaggacuauccugcugccaagagggucaaguuggacagugucagaguccugagacagaucagcaacaaccgaaaaugcaccagccccagguccucggacaccgaggagaaugucaagaggcgaacacacaacgucuuggagcgccagaggaggaacgagcuaaaacggagcuuuuuugcccugcgugaccagaucccggaguuggaaaacaaugaaaaggcccccaagguaguuauccuuaaaaaagccacagcauacauccuguccguccaagcagaggagcaaaagcucauuucugaagaggacuuguugcggaaacgacgagaacaguugaaacacaaacuugaacagcuacggaacucuugugcguaa

SEQ ID NO: 16 - RNA, 2181 nt, Artificial Sequence
  Cyclin T1 - pseudouridine* (Denoted by P)
  Pseudouridine (1)..(2181): n denotes pseudouridine
  misc_feature (2)..(2): n is a, c, g, or u
  misc_feature (34)..(34): n is a, c, g, or u
  misc_feature (37)..(37): n is a, c, g, or u
  misc_feature (39)..(41): n is a, c, g, or u
  misc_feature (45)..(45): n is a, c, g, or u
  misc_feature (56)..(56): n is a, c, g, or u
  misc_feature (63)..(63): n is a, c, g, or u
  misc_feature (70)..(70): n is a, c, g, or u
  misc_feature (75)..(75): n is a, c, g, or u
  misc_feature (78)..(81): n is a, c, g, or u
  misc_feature (86)..(86): n is a, c, g, or u
  misc_feature (96)..(96): n is a, c, g, or u
  misc_feature (104)..(106): n is a, c, g, or u
  misc_feature (108)..(109): n is a, c, g, or u
  misc_feature (111)..(111): n is a, c, g, or u
  misc_feature (129)..(129): n is a, c, g, or u
  misc_feature (131)..(131): n is a, c, g, or u
  misc_feature (134)..(135): n is a, c, g, or u
  misc_feature (143)..(143): n is a, c, g, or u
  misc_feature (153)..(153): n is a, c, g, or u
  misc_feature (155)..(156): n is a, c, g, or u
  misc_feature (161)..(161): n is a, c, g, or u
  misc_feature (163)..(163): n is a, c, g, or u
  misc_feature (169)..(170): n is a, c, g, or u
  misc_feature (174)..(174): n is a, c, g, or u
  misc_feature (176)..(176): n is a, c, g, or u
  misc_feature (183)..(183): n is a, c, g, or u
  misc_feature (186)..(186): n is a, c, g, or u
  misc_feature (188)..(188): n is a, c, g, or u
  misc_feature (191)..(191): n is a, c, g, or u
  misc_feature (193)..(193): n is a, c, g, or u
  misc_feature (197)..(197): n is a, c, g, or u
  misc_feature (201)..(201): n is a, c, g, or u
  misc_feature (205)..(206): n is a, c, g, or u
  misc_feature (208)..(208): n is a, c, g, or u
  misc_feature (212)..(212): n is a, c, g, or u
  misc_feature (215)..(216): n is a, c, g, or u
  misc_feature (220)..(220): n is a, c, g, or u
  misc_feature (223)..(224): n is a, c, g, or u
  misc_feature (232)..(233): n is a, c, g, or u
  misc_feature (237)..(237): n is a, c, g, or u
  misc_feature (243)..(244): n is a, c, g, or u
  misc_feature (246)..(246): n is a, c, g, or u
  misc_feature (248)..(248): n is a, c, g, or u
  misc_feature (252)..(252): n is a, c, g, or u
  misc_feature (262)..(263): n is a, c, g, or u
  misc_feature (265)..(267): n is a, c, g, or u
  misc_feature (269)..(269): n is a, c, g, or u
  misc_feature (276)..(276): n is a, c, g, or u
  misc_feature (281)..(281): n is a, c, g, or u
  misc_feature (301)..(302): n is a, c, g, or u
  misc_feature (309)..(309): n is a, c, g, or u
  misc_feature (311)..(311): n is a, c, g, or u
  misc_feature (314)..(314): n is a, c, g, or u
  misc_feature (320)..(320): n is a, c, g, or u
  misc_feature (327)..(327): n is a, c, g, or u
  misc_feature (330)..(331): n is a, c, g, or u
  misc_feature (333)..(333): n is a, c, g, or u
  misc_feature (335)..(335): n is a, c, g, or u
  misc_feature (339)..(339): n is a, c, g, or u
  misc_feature (342)..(342): n is a, c, g, or u
  misc_feature (349)..(349): n is a, c, g, or u
  misc_feature (353)..(354): n is a, c, g, or u
  misc_feature (357)..(357): n is a, c, g, or u
  misc_feature (360)..(360): n is a, c, g, or u
  misc_feature (363)..(363): n is a, c, g, or u
  misc_feature (369)..(369): n is a, c, g, or u
  misc_feature (375)..(376): n is a, c, g, or u
  misc_feature (378)..(380): n is a, c, g, or u
  misc_feature (389)..(390): n is a, c, g, or u
  misc_feature (396)..(396): n is a, c, g, or u
  misc_feature (398)..(398): n is a, c, g, or u
  misc_feature (401)..(401): n is a, c, g, or u
  misc_feature (404)..(407): n is a, c, g, or u
  misc_feature (416)..(416): n is a, c, g, or u
  misc_feature (419)..(422): n is a, c, g, or u
  misc_feature (429)..(431): n is a, c, g, or u
  misc_feature (436)..(438): n is a, c, g, or u
  misc_feature (443)..(443): n is a, c, g, or u
  misc_feature (449)..(450): n is a, c, g, or u
  misc_feature (453)..(453): n is a, c, g, or u
  misc_feature (462)..(462): n is a, c, g, or u
  misc_feature (465)..(465): n is a, c, g, or u
  misc_feature (468)..(468): n is a, c, g, or u
  misc_feature (470)..(470): n is a, c, g, or u
  misc_feature (473)..(473): n is a, c, g, or u
  misc_feature (478)..(478): n is a, c, g, or u
  misc_feature (483)..(483): n is a, c, g, or u
  misc_feature (488)..(489): n is a, c, g, or u
  misc_feature (491)..(492): n is a, c, g, or u
  misc_feature (508)..(509): n is a, c, g, or u
  misc_feature (519)..(520): n is a, c, g, or u
  misc_feature (522)..(523): n is a, c, g, or u
  misc_feature (526)..(527): n is a, c, g, or u
  misc_feature (530)..(530): n is a, c, g, or u
  misc_feature (545)..(545): n is a, c, g, or u
  misc_feature (549)..(551): n is a, c, g, or u
  misc_feature (559)..(561): n is a, c, g, or u
  misc_feature (566)..(566): n is a, c, g, or u
  misc_feature (571)..(571): n is a, c, g, or u
  misc_feature (579)..(579): n is a, c, g, or u
  misc_feature (582)..(582): n is a, c, g, or u
  misc_feature (584)..(584): n is a, c, g, or u
  misc_feature (587)..(587): n is a, c, g, or u
  misc_feature (592)..(592): n is a, c, g, or u
  misc_feature (594)..(594): n is a, c, g, or u
  misc_feature (596)..(596): n is a, c, g, or u
  misc_feature (598)..(598): n is a, c, g, or u
  misc_feature (602)..(603): n is a, c, g, or u
  misc_feature (608)..(608): n is a, c, g, or u
  misc_feature (612)..(613): n is a, c, g, or u
  misc_feature (619)..(619): n is a, c, g, or u
  misc_feature (622)..(622): n is a, c, g, or u
  misc_feature (627)..(628): n is a, c, g, or u
  misc_feature (635)..(635): n is a, c, g, or u
  misc_feature (641)..(641): n is a, c, g, or u
  misc_feature (643)..(643): n is a, c, g, or u
  misc_feature (648)..(648): n is a, c, g, or u
  misc_feature (661)..(661): n is a, c, g, or u
  misc_feature (664)..(664): n is a, c, g, or u
  misc_feature (670)..(670): n is a, c, g, or u
  misc_feature (672)..(672): n is a, c, g, or u
  misc_feature (674)..(675): n is a, c, g, or u
  misc_feature (684)..(684): n is a, c, g, or u
  misc_feature (686)..(686): n is a, c, g, or u
  misc_feature (691)..(692): n is a, c, g, or u
  misc_feature (698)..(701): n is a, c, g, or u
  misc_feature (705)..(705): n is a, c, g, or u
  misc_feature (710)..(710): n is a, c, g, or u
  misc_feature (717)..(717): n is a, c, g, or u
  misc_feature (721)..(723): n is a, c, g, or u
  misc_feature (725)..(725): n is a, c, g, or u
  misc_feature (731)..(734): n is a, c, g, or u
  misc_feature (744)..(744): n is a, c, g, or u
  misc_feature (755)..(755): n is a, c, g, or u
  misc_feature (764)..(766): n is a, c, g, or u
  misc_feature (771)..(772): n is a, c, g, or u
  misc_feature (781)..(781): n is a, c, g, or u
  misc_feature (789)..(789): n is a, c, g, or u
  misc_feature (810)..(810): n is a, c, g, or u
  misc_feature (825)..(825): n is a, c, g, or u
  misc_feature (834)..(835): n is a, c, g, or u
  misc_feature (848)..(848): n is a, c, g, or u
  misc_feature (851)..(851): n is a, c, g, or u
  misc_feature (855)..(855): n is a, c, g, or u
  misc_feature (857)..(857): n is a, c, g, or u
  misc_feature (860)..(862): n is a, c, g, or u
  misc_feature (871)..(871): n is a, c, g, or u
  misc_feature (873)..(874): n is a, c, g, or u
  misc_feature (887)..(888): n is a, c, g, or u
  misc_feature (894)..(896): n is a, c, g, or u
  misc_feature (899)..(899): n is a, c, g, or u
  misc_feature (905)..(905): n is a, c, g, or u
  misc_feature (907)..(907): n is a, c, g, or u
  misc_feature (912)..(913): n is a, c, g, or u
  misc_feature (915)..(915): n is a, c, g, or u
  misc_feature (924)..(924): n is a, c, g, or u
  misc_feature (929)..(929): n is a, c, g, or u
  misc_feature (933)..(934): n is a, c, g, or u
  misc_feature (938)..(938): n is a, c, g, or u
  misc_feature (944)..(944): n is a, c, g, or u
  misc_feature (946)..(946): n is a, c, g, or u
  misc_feature (955)..(955): n is a, c, g, or u
  misc_feature (958)..(958): n is a, c, g, or u
  misc_feature (967)..(968): n is a, c, g, or u
  misc_feature (975)..(975): n is a, c, g, or u
  misc_feature (977)..(977): n is a, c, g, or u
  misc_feature (983)..(983): n is a, c, g, or u
  misc_feature (985)..(986): n is a, c, g, or u
  misc_feature (999)..(1000): n is a, c, g, or u
  misc_feature (1004)..(1004): n is a, c, g, or u
  misc_feature (1006)..(1006): n is a, c, g, or u
  misc_feature (1009)..(1009): n is a, c, g, or u
  misc_feature (1017)..(1018): n is a, c, g, or u
  misc_feature (1020)..(1022): n is a, c, g, or u
  misc_feature (1028)..(1028): n is a, c, g, or u
  misc_feature (1035)..(1035): n is a, c, g, or u
  misc_feature (1038)..(1038): n is a, c, g, or u
  misc_feature (1044)..(1044): n is a, c, g, or u
  misc_feature (1047)..(1047): n is a, c, g, or u
  misc_feature (1053)..(1053): n is a, c, g, or u
  misc_feature (1056)..(1056): n is a, c, g, or u
  misc_feature (1062)..(1064): n is a, c, g, or u
  misc_feature (1070)..(1071): n is a, c, g, or u
  misc_feature (1079)..(1080): n is a, c, g, or u
  misc_feature (1083)..(1083): n is a, c, g, or u
  misc_feature (1086)..(1087): n is a, c, g, or u
  misc_feature (1090)..(1091): n is a, c, g, or u
  misc_feature (1101)..(1101): n is a, c, g, or u
  misc_feature (1104)..(1105): n is a, c, g, or u
  misc_feature (1110)..(1110): n is a, c, g, or u
  misc_feature (1114)..(1116): n is a, c, g, or u
  misc_feature (1118)..(1120): n is a, c, g, or u
  misc_feature (1134)..(1134): n is a, c, g, or u
  misc_feature (1137)..(1137): n is a, c, g, or u
  misc_feature (1143)..(1143): n is a, c, g, or u
  misc_feature (1145)..(1145): n is a, c, g, or u
  misc_feature (1150)..(1150): n is a, c, g, or u
  misc_feature (1155)..(1155): n is a, c, g, or u
  misc_feature (1160)..(1160): n is a, c, g, or u
  misc_feature (1162)..(1162): n is a, c, g, or u
  misc_feature (1166)..(1166): n is a, c, g, or u
  misc_feature (1174)..(1174): n is a, c, g, or u
  misc_feature (1188)..(1188): n is a, c, g, or u
  misc_feature (1198)..(1199): n is a, c, g, or u
  misc_feature (1203)..(1203): n is a, c, g, or u
  misc_feature (1220)..(1220): n is a, c, g, or u
  misc_feature (1229)..(1229): n is a, c, g, or u
  misc_feature (1239)..(1239): n is a, c, g, or u
  misc_feature (1241)..(1241): n is a, c, g, or u
  misc_feature (1246)..(1246): n is a, c, g, or u
  misc_feature (1252)..(1252): n is a, c, g, or u
  misc_feature (1254)..(1254): n is a, c, g, or u
  misc_feature (1258)..(1258): n is a, c, g, or u
  misc_feature (1260)..(1260): n is a, c, g, or u
  misc_feature (1263)..(1263): n is a, c, g, or u
  misc_feature (1272)..(1272): n is a, c, g, or u
  misc_feature (1274)..(1274): n is a, c, g, or u
  misc_feature (1277)..(1279): n is a, c, g, or u
  misc_feature (1281)..(1281): n is a, c, g, or u
  misc_feature (1284)..(1284): n is a, c, g, or u
  misc_feature (1287)..(1287): n is a, c, g, or u
  misc_feature (1290)..(1290): n is a, c, g, or u
  misc_feature (1296)..(1297): n is a, c, g, or u
  misc_feature (1299)..(1300): n is a, c, g, or u
  misc_feature (1304)..(1304): n is a, c, g, or u
  misc_feature (1307)..(1308): n is a, c, g, or u
  misc_feature (1310)..(1310): n is a, c, g, or u
  misc_feature (1316)..(1316): n is a, c, g, or u
  misc_feature (1322)..(1322): n is a, c, g, or u
  misc_feature (1329)..(1330): n is a, c, g, or u
  misc_feature (1350)..(1353): n is a, c, g, or u
  misc_feature (1355)..(1355): n is a, c, g, or u
  misc_feature (1365)..(1365): n is a, c, g, or u
  misc_feature (1377)..(1377): n is a, c, g, or u
  misc_feature (1379)..(1379): n is a, c, g, or u
  misc_feature (1385)..(1385): n is a, c, g, or u
  misc_feature (1391)..(1391): n is a, c, g, or u
  misc_feature (1397)..(1397): n is a, c, g, or u
  misc_feature (1404)..(1404): n is a, c, g, or u
  misc_feature (1410)..(1410): n is a, c, g, or u
  misc_feature (1416)..(1416): n is a, c, g, or u
  misc_feature (1420)..(1420): n is a, c, g, or u
  misc_feature (1422)..(1423): n is a, c, g, or u
  misc_feature (1439)..(1439): n is a, c, g, or u
  misc_feature (1445)..(1445): n is a, c, g, or u
  misc_feature (1451)..(1451): n is a, c, g, or u
  misc_feature (1457)..(1457): n is a, c, g, or u
  misc_feature (1461)..(1461): n is a, c, g, or u
  misc_feature (1464)..(1464): n is a, c, g, or u
  misc_feature (1470)..(1470): n is a, c, g, or u
  misc_feature (1473)..(1473): n is a, c, g, or u
  misc_feature (1482)..(1483): n is a, c, g, or u
  misc_feature (1485)..(1485): n is a, c, g, or u
  misc_feature (1487)..(1487): n is a, c, g, or u
  misc_feature (1497)..(1497): n is a, c, g, or u
  misc_feature (1499)..(1500): n is a, c, g, or u
  misc_feature (1536)..(1536): n is a, c, g, or u
  misc_feature (1543)..(1543): n is a, c, g, or u
  misc_feature (1545)..(1545): n is a, c, g, or u
  misc_feature (1548)..(1548): n is a, c, g, or u
  misc_feature (1551)..(1551): n is a, c, g, or u
  misc_feature (1554)..(1554): n is a, c, g, or u
  misc_feature (1557)..(1557): n is a, c, g, or u
  misc_feature (1560)..(1560): n is a, c, g, or u
  misc_feature (1563)..(1563): n is a, c, g, or u
  misc_feature (1566)..(1566): n is a, c, g, or u
  misc_feature (1573)..(1573): n is a, c, g, or u
  misc_feature (1585)..(1585): n is a, c, g, or u
  misc_feature (1587)..(1587): n is a, c, g, or u
  misc_feature (1590)..(1591): n is a, c, g, or u
  misc_feature (1598)..(1599): n is a, c, g, or u
  misc_feature (1604)..(1605): n is a, c, g, or u
  misc_feature (1608)..(1608): n is a, c, g, or u
  misc_feature (1611)..(1611): n is a, c, g, or u
  misc_feature (1623)..(1623): n is a, c, g, or u
  misc_feature (1626)..(1626): n is a, c, g, or u
  misc_feature (1629)..(1629): n is a, c, g, or u
  misc_feature (1632)..(1632): n is a, c, g, or u
  misc_feature (1641)..(1641): n is a, c, g, or u
  misc_feature (1644)..(1644): n is a, c, g, or u
  misc_feature (1660)..(1661): n is a, c, g, or u
  misc_feature (1668)..(1668): n is a, c, g, or u
  misc_feature (1675)..(1675): n is a, c, g, or u
  misc_feature (1677)..(1677): n is a, c, g, or u
  misc_feature (1681)..(1682): n is a, c, g, or u
  misc_feature (1684)..(1684): n is a, c, g, or u
  misc_feature (1686)..(1686): n is a, c, g, or u
  misc_feature (1689)..(1690): n is a, c, g, or u
  misc_feature (1692)..(1696): n is a, c, g, or u
  misc_feature (1699)..(1699): n is a, c, g, or u
  misc_feature (1701)..(1702): n is a, c, g, or u
  misc_feature (1707)..(1708): n is a, c, g, or u
  misc_feature (1710)..(1710): n is a, c, g, or u
  misc_feature (1713)..(1713): n is a, c, g, or u
  misc_feature (1716)..(1716): n is a, c, g, or u
  misc_feature (1729)..(1729): n is a, c, g, or u
  misc_feature (1731)..(1731): n is a, c, g, or u
  misc_feature (1740)..(1740): n is a, c, g, or u
  misc_feature (1749)..(1749): n is a, c, g, or u
  misc_feature (1751)..(1751): n is a, c, g, or u
  misc_feature (1753)..(1755): n is a, c, g, or u
  misc_feature (1758)..(1758): n is a, c, g, or u
  misc_feature (1761)..(1761): n is a, c, g, or u
  misc_feature (1772)..(1773): n is a, c, g, or u
  misc_feature (1782)..(1782): n is a, c, g, or u
  misc_feature (1785)..(1785): n is a, c, g, or u
  misc_feature (1789)..(1789): n is a, c, g, or u
  misc_feature (1792)..(1792): n is a, c, g, or u
  misc_feature (1794)..(1795): n is a, c, g, or u
  misc_feature (1799)..(1799): n is a, c, g, or u
  misc_feature (1803)..(1805): n is a, c, g, or u
  misc_feature (1807)..(1807): n is a, c, g, or u
  misc_feature (1810)..(1811): n is a, c, g, or u
  misc_feature (1815)..(1816): n is a, c, g, or u
  misc_feature (1820)..(1821): n is a, c, g, or u
  misc_feature (1824)..(1824): n is a, c, g, or u
  misc_feature (1829)..(1829): n is a, c, g, or u
  misc_feature (1833)..(1833): n is a, c, g, or u
  misc_feature (1838)..(1838): n is a, c, g, or u
  misc_feature (1842)..(1842): n is a, c, g, or u
  misc_feature (1848)..(1848): n is a, c, g, or u
  misc_feature (1852)..(1852): n is a, c, g, or u
  misc_feature (1863)..(1863): n is a, c, g, or u
  misc_feature (1868)..(1870): n is a, c, g, or u
  misc_feature (1873)..(1876): n is a, c, g, or u
  misc_feature (1888)..(1888): n is a, c, g, or u
  misc_feature (1890)..(1890): n is a, c, g, or u
  misc_feature (1896)..(1896): n is a, c, g, or u
  misc_feature (1899)..(1899): n is a, c, g, or u
  misc_feature (1901)..(1901): n is a, c, g, or u
  misc_feature (1905)..(1905): n is a, c, g, or u
  misc_feature (1908)..(1909): n is a, c, g, or u
  misc_feature (1916)..(1916): n is a, c, g, or u
  misc_feature (1920)..(1920): n is a, c, g, or u
  misc_feature (1932)..(1932): n is a, c, g, or u
  misc_feature (1941)..(1941): n is a, c, g, or u
  misc_feature (1944)..(1944): n is a, c, g, or u
  misc_feature (1964)..(1964): n is a, c, g, or u
  misc_feature (1969)..(1969): n is a, c, g, or u
  misc_feature (1971)..(1971): n is a, c, g, or u
  misc_feature (1980)..(1980): n is a, c, g, or u
  misc_feature (1982)..(1982): n is a, c, g, or u
  misc_feature (1986)..(1986): n is a, c, g, or u
  misc_feature (1988)..(1988): n is a, c, g, or u
  misc_feature (1991)..(1992): n is a, c, g, or u
  misc_feature (1996)..(1996): n is a, c, g, or u
  misc_feature (2000)..(2000): n is a, c, g, or u
  misc_feature (2003)..(2003): n is a, c, g, or u
  misc_feature (2007)..(2007): n is a, c, g, or u
  misc_feature (2016)..(2016): n is a, c, g, or u
  misc_feature (2018)..(2019): n is a, c, g, or u
  misc_feature (2028)..(2028): n is a, c, g, or u
  misc_feature (2037)..(2037): n is a, c, g, or u
  misc_feature (2041)..(2043): n is a, c, g, or u
  misc_feature (2047)..(2049): n is a, c, g, or u
  misc_feature (2051)..(2052): n is a, c, g, or u
  misc_feature (2055)..(2055): n is a, c, g, or u
  misc_feature (2058)..(2059): n is a, c, g, or u
  misc_feature (2061)..(2061): n is a, c, g, or u
  misc_feature (2064)..(2064): n is a, c, g, or u
  misc_feature (2068)..(2068): n is a, c, g, or u
  misc_feature (2070)..(2070): n is a, c, g, or u
  misc_feature (2072)..(2072): n is a, c, g, or u
  misc_feature (2076)..(2076): n is a, c, g, or u
  misc_feature (2079)..(2079): n is a, c, g, or u
  misc_feature (2083)..(2083): n is a, c, g, or u
  misc_feature (2085)..(2085): n is a, c, g, or u
  misc_feature (2088)..(2088): n is a, c, g, or u
  misc_feature (2093)..(2093): n is a, c, g, or u
  misc_feature (2095)..(2095): n is a, c, g, or u
  misc_feature (2098)..(2098): n is a, c, g, or u
  misc_feature (2104)..(2104): n is a, c, g, or u
  misc_feature (2106)..(2106): n is a, c, g, or u
  misc_feature (2112)..(2112): n is a, c, g, or u
  misc_feature (2136)..(2136): n is a, c, g, or u
  misc_feature (2138)..(2138): n is a, c, g, or u
  misc_feature (2143)..(2143): n is a, c, g, or u
  misc_feature (2151)..(2151): n is a, c, g, or u
  misc_feature (2154)..(2154): n is a, c, g, or u
  misc_feature (2162)..(2163): n is a, c, g, or u
  misc_feature (2171)..(2172): n is a, c, g, or u
  misc_feature (2175)..(2175): n is a, c, g, or u
  misc_feature (2179)..(2179): n is a, c, g, or u
anggagggagagaggaagaacaacaacaaacggnggnannncacncgagaacagcnggaaaanagcccancccgncgnnnnggcgnggacccaganaaagaacnnncnnancgccagcaggcggccaancngcnncaggacanggggcagcgncnnaacgncncacaanngacnancaacacngcnanagnanacangcancganncnacanganncagnccnncacacagnncccnggaaanncngnggcnccagcagccnngnnncnagcagcnaaagnggaggagcagcccaaaaaannggaacangncancaaggnagcacanacnngncnccanccncaggaancccnnccnganacnagaagngaggcnnannngcaacaagnncaagancnggncannnnagaaagcanaannnngcagacnnnaggcnnngaacnaacaanngancacccacanacncangnagnaaagngcacncaacnngnncgagcaagcaaggacnnagcacagacnncnnacnncanggcaaccaacagccngcannngaccacannnagccngcagnacacaccnccngnggnggccngngncngcanncaccnggcnngcaagnggnccaanngggagancccagncncaacngacgggaagcacnggngggagnangnngacgccacngngaccnnggaacnnnnagangaacngacacangagnnncnacagannnnggagaaaacncccaacaggcncaaacgcannnggaannggagggcangcgaggcngccaagaaaacaaaagcagangaccgaggaacagangaaaagacnncagagcagacaanccncaanangannncccagagcncnncagacacaaccanngcaggnnnaangagcangncaacnncnaccacaagngcagngccnncccngccagncnccgaagagncanccagcaacnnaaccagngnggagangnngccgggcaagcgnnggcngnccncccaaccnncnnncaaacnagaaccnacncagggncancggacnagngagaannnagcacnnacaggagnngancannccnnaccacagganggnncaaangcannnannncccagaagcagaanagnaagagngngccancagcnaaagngncacngaaagaanaccgcgcgaagcangcagaagaannggcngcccagaagaggcaacnggagaacanggaagccaangngaagncacaanangcanangcngcccagaancnccnnncncancanganagccanncnncagncanncnaaaaangcccanagagggnncagaaaaccccgagcggccnnnncnggaaaaggcngacaaaacagcncncaaaangagaancccagnggcaggnggaganaaagcngcgncnncaaaaccagaggaganaaaaangcgcanaaaagnccangcngcagcnganaagcacaanncngnagaggacagngnnacaaagagccgagagcacaaagaaaagcacaagacncacccancnaancancancancancanaancaccacncacacaagcacncncanncccaacnnccagnnggnacngggaacaaacgnccnggnganccaaaacanagnagccagacaagcaacnnagcacanaaaaccnanagcnngncnagnncnnnnnccncnnccagnncnacncgnaaaaggggacccncngaagagacnggaggggcngngnnngancanccagccaaganngccaagagnacnaaanccncnncccnaaannncnccnncccnncacnnccnacaangggncagangccngggcanagcncagacacaagnggccnnnccnnnncacagcccagcngnaaaacncgngncccncanncgaaacngganaaagggcccacnggggccaanggncacaacacgacccagacaanagacnancaagacacngngaanangcnncacncccngcncagngcccagggngnncagcccacncagcccacngcannngaannngnncgnccnnanagngacnancngaanccncggncnggnggaancnccncgagancnggcaanacagacaaaccccggccaccaccncngccancagaaccnccnccaccacnnccaccccnnccnaagnaa

SEQ ID NO: 17 - RNA, 1119 nt, Artificial Sequence
  CDK9 - pseudouridine* (Denoted by P)
  Pseudouridine (1)..(1119): n denotes pseudouridine
  misc_feature (2)..(2): n is a, c, g, or u
  misc_feature (13)..(13): n is a, c, g, or u
  misc_feature (19)..(19): n is a, c, g, or u
  misc_feature (23)..(23): n is a, c, g, or u
  misc_feature (28)..(28): n is a, c, g, or u
  misc_feature (33)..(37): n is a, c, g, or u
  misc_feature (39)..(39): n is a, c, g, or u
  misc_feature (42)..(42): n is a, c, g, or u
  misc_feature (47)..(49): n is a, c, g, or u
  misc_feature (55)..(55): n is a, c, g, or u
  misc_feature (65)..(65): n is a, c, g, or u
  misc_feature (74)..(74): n is a, c, g, or u
  misc_feature (88)..(89): n is a, c, g, or u
  misc_feature (98)..(98): n is a, c, g, or u
  misc_feature (100)..(101): n is a, c, g, or u
  misc_feature (134)..(134): n is a, c, g, or u
  misc_feature (138)..(138): n is a, c, g, or u
  misc_feature (140)..(140): n is a, c, g, or u
  misc_feature (149)..(149): n is a, c, g, or u
  misc_feature (152)..(152): n is a, c, g, or u
  misc_feature (155)..(155): n is a, c, g, or u
  misc_feature (175)..(176): n is a, c, g, or u
  misc_feature (182)..(183): n is a, c, g, or u
  misc_feature (190)..(191): n is a, c, g, or u
  misc_feature (200)..(200): n is a, c, g, or u
  misc_feature (206)..(206): n is a, c, g, or u
  misc_feature (209)..(210): n is a, c, g, or u
  misc_feature (215)..(216): n is a, c, g, or u
  misc_feature (218)..(218): n is a, c, g, or u
  misc_feature (231)..(231): n is a, c, g, or u
  misc_feature (233)..(233): n is a, c, g, or u
  misc_feature (236)..(236): n is a, c, g, or u
  misc_feature (241)..(242): n is a, c, g, or u
  misc_feature (245)..(246): n is a, c, g, or u
  misc_feature (251)..(253): n is a, c, g, or u
  misc_feature (255)..(255): n is a, c, g, or u
  misc_feature (267)..(268): n is a, c, g, or u
  misc_feature (274)..(274): n is a, c, g, or u
  misc_feature (276)..(276): n is a, c, g, or u
  misc_feature (283)..(283): n is a, c, g, or u
  misc_feature (291)..(291): n is a, c, g, or u
  misc_feature (294)..(294): n is a, c, g, or u
  misc_feature (296)..(296): n is a, c, g, or u
  misc_feature (298)..(298): n is a, c, g, or u
  misc_feature (302)..(302): n is a, c, g, or u
  misc_feature (305)..(305): n is a, c, g, or u
  misc_feature (307)..(308): n is a, c, g, or u
  misc_feature (313)..(314): n is a, c, g, or u
  misc_feature (316)..(316): n is a, c, g, or u
  misc_feature (324)..(324): n is a, c, g, or u
  misc_feature (329)..(330): n is a, c, g, or u
  misc_feature (333)..(333): n is a, c, g, or u
  misc_feature (338)..(338): n is a, c, g, or u
  misc_feature (340)..(341): n is a, c, g, or u
  misc_feature (348)..(348): n is a, c, g, or u
  misc_feature (350)..(353): n is a, c, g, or u
  misc_feature (356)..(356): n is a, c, g, or u
  misc_feature (361)..(362): n is a, c, g, or u
  misc_feature (368)..(368): n is a, c, g, or u
  misc_feature (370)..(370): n is a, c, g, or u
  misc_feature (372)..(372): n is a, c, g, or u
  misc_feature (377)..(377): n is a, c, g, or u
  misc_feature (386)..(386): n is a, c, g, or u
  misc_feature (389)..(389): n is a, c, g, or u
  misc_feature (395)..(395): n is a, c, g, or u
  misc_feature (398)..(398): n is a, c, g, or u
  misc_feature (401)..(402): n is a, c, g, or u
  misc_feature (410)..(410): n is a, c, g, or u
  misc_feature (412)..(412): n is a, c, g, or u
  misc_feature (415)..(415): n is a, c, g, or u
  misc_feature (419)..(419): n is a, c, g, or u
  misc_feature (434)..(434): n is a, c, g, or u
  misc_feature (437)..(437): n is a, c, g, or u
  misc_feature (441)..(441): n is a, c, g, or u
  misc_feature (449)..(449): n is a, c, g, or u
  misc_feature (456)..(456): n is a, c, g, or u
  misc_feature (459)..(459): n is a, c, g, or u
  misc_feature (462)..(462): n is a, c, g, or u
  misc_feature (464)..(464): n is a, c, g, or u
  misc_feature (467)..(468): n is a, c, g, or u
  misc_feature (470)..(470): n is a, c, g, or u
  misc_feature (474)..(474): n is a, c, g, or u
  misc_feature (477)..(477): n is a, c, g, or u
  misc_feature (480)..(480): n is a, c, g, or u
  misc_feature (485)..(485): n is a, c, g, or u
  misc_feature (488)..(488): n is a, c, g, or u
  misc_feature (494)..(494): n is a, c, g, or u
  misc_feature (502)..(504): n is a, c, g, or u
  misc_feature (509)..(509): n is a, c, g, or u
  misc_feature (520)..(521): n is a, c, g, or u
  misc_feature (527)..(527): n is a, c, g, or u
  misc_feature (553)..(553): n is a, c, g, or u
  misc_feature (564)..(564): n is a, c, g, or u
  misc_feature (566)..(566): n is a, c, g, or u
  misc_feature (569)..(569): n is a, c, g, or u
  misc_feature (575)..(575): n is a, c, g, or u
  misc_feature (577)..(577): n is a, c, g, or u
  misc_feature (580)..(580): n is a, c, g, or u
  misc_feature (596)..(596): n is a, c, g, or u
  misc_feature (598)..(599): n is a, c, g, or u
  misc_feature (602)..(602): n is a, c, g, or u
  misc_feature (616)..(616): n is a, c, g, or u
  misc_feature (629)..(630): n is a, c, g, or u
  misc_feature (635)..(635): n is a, c, g, or u
  misc_feature (637)..(637): n is a, c, g, or u
  misc_feature (642)..(642): n is a, c, g, or u
  misc_feature (645)..(645): n is a, c, g, or u
  misc_feature (649)..(649): n is a, c, g, or u
  misc_feature (653)..(653): n is a, c, g, or u
  misc_feature (656)..(656): n is a, c, g, or u
  misc_feature (665)..(665): n is a, c, g, or u
  misc_feature (667)..(667): n is a, c, g, or u
  misc_feature (683)..(683): n is a, c, g, or u
  misc_feature (686)..(686): n is a, c, g, or u
  misc_feature (713)..(713): n is a, c, g, or u
  misc_feature (719)..(719): n is a, c, g, or u
  misc_feature (722)..(722): n is a, c, g, or u
  misc_feature (726)..(726): n is a, c, g, or u
  misc_feature (731)..(731): n is a, c, g, or u
  misc_feature (733)..(733): n is a, c, g, or u
  misc_feature (739)..(739): n is a, c, g, or u
  misc_feature (743)..(743): n is a, c, g, or u
  misc_feature (750)..(750): n is a, c, g, or u
  misc_feature (755)..(755): n is a, c, g, or u
  misc_feature (757)..(757): n is a, c, g, or u
  misc_feature (767)..(767): n is a, c, g, or u
  misc_feature (775)..(775): n is a, c, g, or u
  misc_feature (777)..(777): n is a, c, g, or u
  misc_feature (782)..(782): n is a, c, g, or u
  misc_feature (784)..(784): n is a, c, g, or u
  misc_feature (794)..(794): n is a, c, g, or u
  misc_feature (800)..(800): n is a, c, g, or u
  misc_feature (803)..(803): n is a, c, g, or u
  misc_feature (824)..(824): n is a, c, g, or u
  misc_feature (836)..(836): n is a, c, g, or u
  misc_feature (844)..(844): n is a, c, g, or u
  misc_feature (846)..(846): n is a, c, g, or u
  misc_feature (848)..(848): n is a, c, g, or u
  misc_feature (852)..(852): n is a, c, g, or u
  misc_feature (859)..(859): n is a, c, g, or u
  misc_feature (866)..(866): n is a, c, g, or u
  misc_feature (872)..(872): n is a, c, g, or u
  misc_feature (875)..(875): n is a, c, g, or u
  misc_feature (884)..(884): n is a, c, g, or u
  misc_feature (887)..(887): n is a, c, g, or u
  misc_feature (890)..(890): n is a, c, g, or u
  misc_feature (893)..(893): n is a, c, g, or u
  misc_feature (900)..(900): n is a, c, g, or u
  misc_feature (911)..(911): n is a, c, g, or u
  misc_feature (921)..(921): n is a, c, g, or u
  misc_feature (929)..(929): n is a, c, g, or u
  misc_feature (940)..(941): n is a, c, g, or u
  misc_feature (943)..(944): n is a, c, g, or u
  misc_feature (946)..(946): n is a, c, g, or u
  misc_feature (949)..(949): n is a, c, g, or u
  misc_feature (959)..(959): n is a, c, g, or u
  misc_feature (964)..(964): n is a, c, g, or u
  misc_feature (971)..(971): n is a, c, g, or u
  misc_feature (980)..(980): n is a, c, g, or u
  misc_feature (983)..(983): n is a, c, g, or u
  misc_feature (985)..(985): n is a, c, g, or u
  misc_feature (995)..(995): n is a, c, g, or u
  misc_feature (1000)..(1000): n is a, c, g, or u
  misc_feature (1004)..(1004): n is a, c, g, or u
  misc_feature (1006)..(1007): n is a, c, g, or u
  misc_feature (1012)..(1012): n is a, c, g, or u
  misc_feature (1015)..(1016): n is a, c, g, or u
  misc_feature (1046)..(1046): n is a, c, g, or u
  misc_feature (1057)..(1057): n is a, c, g, or u
  misc_feature (1071)..(1071): n is a, c, g, or u
  misc_feature (1077)..(1077): n is a, c, g, or u
  misc_feature (1102)..(1104): n is a, c, g, or u
  misc_feature (1112)..(1112): n is a, c, g, or u
  misc_feature (1114)..(1115): n is a, c, g, or u
  misc_feature (1117)..(1117): n is a, c, g, or u
anggcaaagcagnacgacncggnggagngcccnnnnngngangaagnnnccaaanacgagaagcncgccaagancggccaaggcaccnncggggaggngnncaaggccaggcaccgcaagaccggccagaaggnggcncngaagaaggngcnganggaaaacgagaaggaggggnnccccannacagccnngcgggagancaaganccnncagcnncnaaaacacgagaangnggncaacnnganngagannngncgaaccaaagcnncccccnanaaccgcngcaagggnagnananaccnggngnncgacnncngcgagcangaccnngcngggcngnngagcaangnnnnggncaagnncacgcngncngagancaagagggngangcagangcngcnnaacggccncnacnacanccacagaaacaaganccngcanagggacangaaggcngcnaangngcnnancacncgnganggggnccngaagcnggcagacnnngggcnggcccgggccnncagccnggccaagaacagccagcccaaccgcnacaccaaccgngnggngacacncnggnaccggcccccggagcngnngcncggggagcgggacnacggcccccccanngaccngnggggngcngggngcancanggcagagangnggacccgcagccccancangcagggcaacacggagcagcaccaacncgcccncancagncagcncngcggcnccancaccccngaggngnggccaaacgnggacaacnangagcngnacgaaaagcnggagcnggncaagggccagaagcggaaggngaaggacaggcngaaggccnangngcgngacccanacgcacnggaccncancgacaagcngcnggngcnggacccngcccagcgcancgacagcgangacgcccncaaccacgacnncnncnggnccgaccccangcccnccgaccncaagggcangcncnccacccaccngacgnccangnncgagnacnnggcaccaccgcgccggaagggcagccagancacccagcagnccaccaaccagagncgcaancccgccaccaccaaccagacggagnnngagcgcgncnncnga

SEQ ID NO: 18 - protein, 580 aa, Artificial Sequence
  cyclin K
MKENKENSSPSVTSANLDHTKPCWYWDKKDLAHTPSQLEGLDPATEARYRREGARFIFDVGTRLGLHYDTLATGIIYFHRFYMFHSFKQFPRYVTGACCLFLAGKVEETPKKCKDIIKTARSLLNDVQFGQFGDDPKEEVMVLERILLQTIKFDLQVEHPYQFLLKYAKQLKGDKNKIQKLVQMAWTFVNDSLCTTLSLQWEPEIIAVAVMYLAGRLCKFEIQEWTSKPMYRRWWEQFVQDVPVDVLEDICHQILDLYSQGKQQMPHHTPHQLQQPPSLQPTPQVPQVQQSQPSQSSEPSQPQQKDPQQPAQQQQPAQQPKKPSPQPSSPRQVKRAVVVSPKEENKAAEPPPPKIPKIETTHPPLPPAHPPPDRKPPLAAALGEAEPPGPVDATDLPKVQIPPPAHPAPVHQPPPLPHRPPPPPPSSYMTGMSTTSSYMSGEGYQSLQSMMKTEGPSYGALPPAYGPPAHLPYHPHVYPPNPPPPPVPPPPASFPPPAIPPPTPGYPPPPPTYNPNFPPPPPRLPPTHAVPPHPPPGLGLPPASYPPPAVPPGGQPPVPPPIPPPGMPPVGGLGRAAWMR

SEQ ID NO: 19 - DNA, 1743 bp, Artificial Sequence
  cyclin K
atgaaggagaataaagaaaattcaagcccttcagtaacttcagcaaacctggaccacacaaagccatgttggtactgggataagaaagacttggctcatacaccctcacaacttgaaggacttgatccagccaccgaggcccggtaccgccgagagggcgctcggttcatctttgatgtgggcacacgtttggggctacactatgataccctggcaactggaataatttattttcatcgcttctatatgtttcattccttcaagcaattcccaagatatgtgacaggagcctgttgcctctttctggctgggaaagtagaagaaacaccaaaaaaatgtaaagatatcatcaaaacagctcgtagtttattaaatgatgtacaatttggccagtttggagatgacccaaaggaggaagtaatggttctggagagaatcttactgcagaccatcaagtttgatttacaggtagaacatccataccagttcctactaaaatatgcaaagcaactcaaaggtgataaaaacaaaattcaaaagttggttcaaatggcatggacatttgtaaatgacagtctctgcaccaccttgtcactgcagtgggaaccagagatcatagcagtagcagtgatgtatctcgcaggacgtttgtgcaaatttgaaatacaagaatggacctccaaacccatgtataggagatggtgggagcagtttgttcaagatgtcccggtcgacgttttggaagacatctgccaccaaatcctggatctttactcacaaggaaaacaacagatgcctcatcacaccccccatcagctgcaacagcccccatctcttcagcctacaccacaagtgccgcaagtacagcagtcacagccgtctcaaagctccgaaccatcccagccccagcagaaggacccccagcaaccagcccagcagcagcagccagcccaacagcccaagaaaccctctccgcagcccagttctccccgacaggttaagcgagccgtggttgtttctcccaaagaagagaacaaagcagcagaaccaccaccacctaaaatccccaaaattgagaccactcatccaccgttgcctccagcccacccacctccagaccggaagcctcccctcgctgctgccttaggtgaggctgagccgccgggccctgtggatgccactgacctccccaaagtccagattccccctccggcccacccggcccctgtgcaccagccaccgccgctgccacaccggcccccgcccccacccccctccagctacatgaccgggatgtccaccaccagctcctacatgtctggagagggctaccagagcctgcagtccatgatgaagaccgagggaccctcctacggtgccctgccccccgcctacggcccacctgcacacctgccctaccacccccatgtctacccgcccaacccgcccccgccacctgtgcctcctcccccagcctccttccccccacctgccatcccaccccctactcctggctaccccccacccccacccacctacaaccccaacttcccacccccacccccacgcctcccgcctacccacgcagtcccccctcatcctcctccagggttgggcctgccgccagccagctacccacctcctgccgtcccccctggaggacagcctcctgtgcccccgcccattcccccacccggcatgcctccagttggggggctggggcgggcagcctggatgagataa

SEQ ID NO: 20 - protein, 730 aa, Artificial Sequence
  cyclin T2
MASGRGASSRWFFTREQLENTPSRRCGVEADKELSCRQQAANLIQEMGQRLNVSQLTINTAIVYMHRFYMHHSFTKFNKNIISSTALFLAAKVEEQARKLEHVIKVAHACLHPLEPLLDTKCDAYLQQTQELVILETIMLQTLGFEITIEHPHTDVVKCTQLVRASKDLAQTSYFMATNSLHLTTFCLQYKPTVIACVCIHLACKWSNWEIPVSTDGKHWWEYVDPTVTLELLDELTHEFLQILEKTPNRLKKIRNWRANQAARKPKVDGQVSETPLLGSSLVQNSILVDSVTGVPTNPSFQKPSTSAFPAPVPLNSGNISVQDSHTSDNLSMLATGMPSTSYGLSSHQEWPQHQDSARTEQLYSQKQETSLSGSQYNINFQQGPSISLHSGLHHRPDKISDHSSVKQEYTHKAGSSKHHGPISTTPGIIPQKMSLDKYREKRKLETLDLDVRDHYIAAQVEQQHKQGQSQAASSSSVTSPIKMKIPIANTEKYMADKKEKSGSLKLRIPIPPTDKSASKEELKMKIKVSSSERHSSSDEGSGKSKHSSPHISRDHKEKHKEHPSSRHHTSSHKHSHSHSGSSSGGSKHSADGIPPTVLRSPVGLSSDGISSSSSSSRKRLHVNDASHNHHSKMSKSSKSSGSSSSSSSSVKQYISSHNSVFNHPLPPPPPVTYQVGYGHLSTLVKLDKKPVETNGPDANHEYSTSSQHMDYKDTFDMLDSLLSAQGMNM

SEQ ID NO: 21 - DNA, 2193 bp, Artificial Sequence
  cyclin T2
atggcgtcgggccgtggagcttcttctcgctggttctttactcgggaacagctggagaacacgccgagccgccgctgcggagtggaggcggataaagagctctcgtgccgccagcaggcggccaacctcatccaggagatgggacagcgtctcaatgtctctcagcttacaataaacactgcgattgtttatatgcacaggttttatatgcaccattctttcaccaaattcaacaaaaatataatatcgtctactgcattatttttggctgcaaaagtggaagaacaggctcgaaaacttgaacatgttatcaaagtagcacatgcttgtcttcatcctctagagccactgctggatactaaatgtgatgcttaccttcaacagactcaagaactggttatacttgaaaccataatgctacaaactctaggttttgagatcaccattgaacacccacacacagatgtggtgaaatgtacccagttagtaagagcaagcaaggatttggcacagacatcctatttcatggctaccaacagtctgcatcttacaaccttctgtcttcagtacaaaccaacagtgatagcatgtgtatgcattcatttggcttgcaaatggtccaattgggagatccctgtatcaactgatggaaagcattggtgggaatatgtggatcctacagttactctagaattattagatgagctaacacatgagtttctacaaatattggagaaaacgcctaataggttgaagaagattcgaaactggagggctaatcaggcagctaggaaaccaaaagtagatggacaggtatcagagacaccacttcttggttcatctttggtccagaattccattttagtagatagtgtcactggtgtgcctacaaacccaagttttcagaaaccatctacatcagcattccctgcgccagtacctctaaattcaggaaatatttctgttcaagacagccatacatctgataatttgtcaatgctagcaacaggaatgccaagtacttcatacggtttatcatcacaccaggaatggcctcaacatcaagactcagcaaggacagaacagctatattcacagaaacaggagacatctttgtctggtagccagtacaacatcaacttccagcagggaccttctatatcactgcattcaggattacatcacagacctgacaaaatttcagatcattcttctgttaagcaagaatatactcataaagcagggagcagtaaacaccatgggccaatttccactactccaggaataattcctcagaaaatgtctttagataaatatagagaaaagcgtaaactagaaactcttgatctcgatgtaagggatcattatatagctgcccaggtagaacagcagcacaaacaagggcagtcacaggcagccagcagcagttctgttacttctcccattaaaatgaaaatacctatcgcaaatactgaaaaatacatggcagacaaaaaggaaaagagtgggtcactgaaattacggattccaataccacccactgataaaagcgccagtaaagaagaactgaaaatgaaaataaaagtttcttcttcagaaagacacagctcttctgatgaaggcagtgggaagagcaaacattcaagcccacatattagcagagaccataaggagaagcacaaggagcatccttcaagccgccaccacaccagcagccacaagcattcccactcgcatagtggcagcagcagcggtggcagtaaacacagtgccgacggaataccacccactgttctgaggagtcctgttggcctgagcagtgatggcatttcctctagctccagctcttcaaggaagaggctgcatgtcaatgatgcatctcacaaccaccactccaaaatgagcaaaagttccaaaagttcaggtagttcatctagttcttcctcctctgttaagcagtatatatcctctcacaactctgtttttaaccatcccttaccccctcctccccctgtcacataccaggtgggctacggacatctcagcaccctcgtgaaactggacaagaagccagtggagaccaacggtcctgatgccaatcacgagtacagtacaagcagccagcatatggactacaaagacacattcgacatgctggactcactgttaagtgcccaaggaatgaacatgtaa

SEQ ID NO: 22 - DNA, 1185 bp, Artificial Sequence
  l-myc
atgtgcgtgtgtgctggctgccgggctgccccgagccggcggggagccggtccgctccaggtggcgggcggctggagcgagggagcggacatggactacgactcgtaccagcactatttctacgactatgactgcggggaggatttctaccgctccacggcgcccagcgaggacatctggaagaaattcgagctggtgccatcgccccccacgtcgccgccctggggcttgggtcccggcgcaggggacccggcccccgggattggtcccccggagccgtggcccggagggtgcaccggagacgaagcggaatcccggggccactcgaaaggctggggcaggaactacgcctccatcatacgccgtgactgcatgtggagcggcttctcggcccgggaacggctggagagagctgtgagcgaccggctcgctcctggcgcgccccgggggaacccgcccaaggcgtccgccgccccggactgcactcccagcctcgaagccggcaacccggcgcccgccgccccctgtccgctgggcgaacccaagacccaggcctgctccgggtccgagagcccaagcgactcggagaatgaagaaattgatgttgtgacagtagagaagaggcagtctctgggtattcggaagccggtcaccatcacggtgcgagcagaccccctggatccctgcatgaagcatttccacatctccatccatcagcaacagcacaactatgctgcccgttttcctccagaaagctgctcccaagaagaggcttcagagaggggtccccaagaagaggttctggagagagatgctgcaggggaaaaggaagatgaggaggatgaagagattgtgagtcccccacctgtagaaagtgaggctgcccagtcctgccaccccaaacctgtcagttctgatactgaggatgtgaccaagaggaagaatcacaacttcctggagcgcaagaggcggaatgacctgcgttcgcgattcttggcgctgagggaccaggtgcccaccctggccagctgctccaaggcccccaaagtagtgatcctaagcaaggccttggaatacttgcaagccctggtgggggctgagaagaggatggctacagagaaaagacagctccgatgccggcagcagcagttgcagaaaagaattgcatacctcactggctactaa

SEQ ID NO: 23 - protein, 394 aa, Artificial Sequence
  l-myc
MCVCAGCRAAPSRRGAGPLQVAGGWSEGADMDYDSYQHYFYDYDCGEDFYRSTAPSEDIWKKFELVPSPPTSPPWGLGPGAGDPAPGIGPPEPWPGGCTGDEAESRGHSKGWGRNYASIIRRDCMWSGFSARERLERAVSDRLAPGAPRGNPPKASAAPDCTPSLEAGNPAPAAPCPLGEPKTQACSGSESPSDSENEEIDVVTVEKRQSLGIRKPVTITVRADPLDPCMKHFHISIHQQQHNYAARFPPESCSQEEASERGPQEEVLERDAAGEKEDEEDEEIVSPPPVESEAAQSCHPKPVSSDTEDVTKRKNHNFLERKRRNDLRSRFLALRDQVPTLASCSKAPKVVILSKALEYLQALVGAEKRMATEKRQLRCRQQQLQKRIAYLTGY

SEQ ID NO: 24 - DNA, 1395 bp, Artificial Sequence
  n-myc
atgccgagctgctccacgtccaccatgccgggcatgatctgcaagaacccagacctcgagtttgactcgctacagccctgcttctacccggacgaagatgacttctacttcggcggccccgactcgacccccccgggggaggacatctggaagaagtttgagctgctgcccacgcccccgctgtcgcccagccgtggcttcgcggagcacagctccgagcccccgagctgggtcacggagatgctgcttgagaacgagctgtggggcagcccggccgaggaggacgcgttcggcctggggggactgggtggcctcacccccaacccggtcatcctccaggactgcatgtggagcggcttctccgcccgcgagaagctggagcgcgccgtgagcgagaagctgcagcacggccgcgggccgccaaccgccggttccaccgcccagtccccgggagccggcgccgccagccctgcgggtcgcgggcacggcggggctgcgggagccggccgcgccggggccgccctgcccgccgagctcgcccacccggccgccgagtgcgtggatcccgccgtggtcttcccctttcccgtgaacaagcgcgagccagcgcccgtgcccgcagccccggccagtgccccggcggcgggccctgcggtcgcctcgggggcgggtattgccgccccagccggggccccgggggtcgcccctccgcgcccaggcggccgccagaccagcggcggcgaccacaaggccctcagtacctccggagaggacaccctgagcgattcagatgatgaagatgatgaagaggaagatgaagaggaagaaatcgacgtggtcactgtggagaagcggcgttcctcctccaacaccaaggctgtcaccacattcaccatcactgtgcgtcccaagaacgcagccctgggtcccgggagggctcagtccagcgagctgatcctcaaacgatgccttcccatccaccagcagcacaactatgccgccccctctccctacgtggagagtgaggatgcacccccacagaagaagataaagagcgaggcgtccccacgtccgctcaagagtgtcatccccccaaaggctaagagcttgagcccccgaaactctgactcggaggacagtgagcgtcgcagaaaccacaacatcctggagcgccagcgccgcaacgaccttcggtccagctttctcacgctcagggaccacgtgccggagttggtaaagaatgagaaggccgccaaggtggtcattttgaaaaaggccactgagtatgtccactccctccaggccgaggagcaccagcttttgctggaaaaggaaaaattgcaggcaagacagcagcagttgctaaagaaaattgaacacgctcggacttgctag

SEQ ID NO: 25 - protein, 464 aa, Artificial Sequence
  n-myc
MPSCSTSTMPGMICKNPDLEFDSLQPCFYPDEDDFYFGGPDSTPPGEDIWKKFELLPTPPLSPSRGFAEHSSEPPSWVTEMLLENELWGSPAEEDAFGLGGLGGLTPNPVILQDCMWSGFSAREKLERAVSEKLQHGRGPPTAGSTAQSPGAGAASPAGRGHGGAAGAGRAGAALPAELAHPAAECVDPAVVFPFPVNKREPAPVPAAPASAPAAGPAVASGAGIAAPAGAPGVAPPRPGGRQTSGGDHKALSTSGEDTLSDSDDEDDEEEDEEEEIDVVTVEKRRSSSNTKAVTTFTITVRPKNAALGPGRAQSSELILKRCLPIHQQHNYAAPSPYVESEDAPPQKKIKSEASPRPLKSVIPPKAKSLSPRNSDSEDSERRRNHNILERQRRNDLRSSFLTLRDHVPELVKNEKAAKVVILKKATEYVHSLQAEEHQLLLEKEKLQARQQQLLKKIEHARTC

SEQ ID NO: 26 - protein, 19 aa, Artificial Sequence
  P2A
ATNFSLLKQAGDVEENPGP

SEQ ID NO: 27 - protein, 20 aa, Artificial Sequence
  E2A
QCTNYALLKLAGDVESNPGP

SEQ ID NO: 28 - protein, 22 aa, Artificial Sequence
  F2A
VKQTLNFDLLKLAGDVESNPGP

SEQ ID NO: 29 - protein, 18 aa, Artificial Sequence
  T2A
EGRGSLLTCGDVEENPGP

SEQ ID NO: 30 - DNA, 19 bp, Artificial Sequence
  guide sequence targeting Larp7
atccggaggaaaaaacctc

SEQ ID NO: 31 - DNA, 19 bp, Artificial Sequence
  guide sequence targeting Larp7
agtctactggagatccaaa

SEQ ID NO: 32 - DNA, 19 bp, Artificial Sequence
  guide sequence targeting Larp7
aagaaaggccgaatgaaaa

SEQ ID NO: 33 - DNA, 19 bp, Artificial Sequence
  guide sequence targeting Larp7
cttacctgaagtcagaaca

SEQ ID NO: 34 - DNA, 19 bp, Artificial Sequence
  guide sequence targeting Larp7
acttttgatcggggagcta

SEQ ID NO: 35 - protein, 589 aa, Artificial Sequence
  Larp7
MIPNIEGMETESGNQEKVMEEESTEKKKEVEKKKRSRVKQVLADIAKQVDFWFGDANLHKDRFLREQIEKSRDGYVDISLLVSFNKMKKLTTDGKLIARALRSSAVVELDLEGTRIRRKKPLGERPKDEDERTVYVELLPKNVNHSWIERVFGKCGNVVYISIPHYKSTGDPKGFAFVEFETKEQAAKAIEFLNNPPEEAPRKPGIFPKTVKNKPIPALRVVEEKKKKKKKKGRMKKEDNIQAKEENMDTSNTSISKMKRSRPTSEGSDIESTEPQKQCSKKKKKRDRVEASSLPEVRTGKRKRSSSEDAESLAPRSKVKKIIQKDIIKEASEASKENRDIEISTEEEKDTGDLKDSSLLKTKRKHKKKHKERHKMGEEVIPLRVLSKSEWMDLKKEYLALQKASMASLKKTISQIKSESEMETDSGVPQNTGMKNEKTANREECRTQEKVNATGPQFVSGVIVKIISTEPLPGRKQVRDTLAAISEVLYVDLLEGDTECHARFKTPEDAQAVINAYTEINKKHCWKLEILSGDHEQRYWQKILVDRQAKLNQPREKKRGTEKLITKAEKIRLAKTQQASKHIRFSEYD

SEQ ID NO: 36 - DNA, 1770 bp, Artificial Sequence
  Larp7
atgatccctaacatagaaggaatggaaactgaaagtggaaatcaggaaaaggtaatggaagaagaaagcactgaaaagaaaaaagaagttgaaaaaaagaaacggtcacgagttaaacaggtgcttgcagatattgctaagcaagtggacttctggtttggggatgcaaatcttcacaaggatagatttcttcgagaacagatagaaaaatctagagatggatatgttgatatatcactacttgtgtcttttaacaaaatgaaaaaattgactactgatgggaagttaattgccagagcattgagaagttcagctgttgtagagcttgatttggaaggcaccagaatccggaggaaaaaacctctgggggaaagaccaaaggatgaggatgaacgcacagtgtatgtggagttacttcccaaaaatgttaatcacagctggattgaaagagtatttgggaaatgtggcaatgttgtttatataagtataccacattataagtctactggagatccaaagggatttgcgtttgtggaatttgaaacaaaagaacaagcagcaaaagcaattgagtttcttaacaacccaccagaagaagcaccaagaaaacctggcatatttcctaaaacagtgaaaaataagcccattccagccttaagagttgtggaagagaagaaaaagaaaaagaagaagaaaggccgaatgaaaaaggaagacaatatccaagccaaagaagaaaacatggacacaagcaacaccagcatcagtaaaatgaaaagatccagacccacatctgagggctctgacattgagtccactgaaccccaaaagcagtgctcaaagaaaaagaaaaaacgggacagagttgaagcatctagcttacctgaagtcagaacagggaagaggaagagaagcagctctgaagatgcagaatccctagctccccgatcaaaagtaaagaaaattattcagaaagacatcattaaggaagcatcagaagcttccaaggaaaatagagatatagaaatctctactgaagaggaaaaggatactggagatctaaaagatagctctctcttgaaaacaaaaaggaaacataagaaaaaacataaagagagacataaaatgggagaagaagttataccattaagagtgctatcaaagagcgaatggatggatttgaaaaaagagtatttagcgctacaaaaagctagcatggcttctttaaaaaaaacaatatcccaaataaaatcagagtcagaaatggaaacagacagtggagtacctcaaaacactggaatgaaaaatgaaaaaacagccaacagggaagagtgtcgcacccaggagaaagttaatgcaacaggaccacagttcgtgagtggagtgattgtgaagatcattagcacagagcctctacctggcaggaaacaagtccgggatactttggcagcaatctcagaagttctttatgttgatttgctagaaggggatacagaatgccatgctagatttaaaactcctgaggatgctcaagcagtaataaatgcctatacagaaattaacaagaaacactgctggaaactcgagatcctttctggtgatcacgaacaaaggtattggcagaagattttggttgatagacaggcaaaacttaatcagcctcgggaaaagaaaagaggcactgaaaagttaatcaccaaagctgaaaagattagactggcaaagactcaacaagcgagtaaacatataagattttctgaatatgattga

SEQ ID NO: 37 - RNA, 1365 nt, Artificial Sequence
  c-Myc - pseudouridine* (Denoted by P)
  Pseudouridine (1)..(1365): n denotes pseudouridine
  misc_feature (2)..(2): n is a, c, g, or u
  misc_feature (6)..(12): n is a, c, g, or u
  misc_feature (17)..(17): n is a, c, g, or u
  misc_feature (20)..(20): n is a, c, g, or u
  misc_feature (36)..(36): n is a, c, g, or u
  misc_feature (47)..(47): n is a, c, g, or u
  misc_feature (53)..(53): n is a, c, g, or u
  misc_feature (59)..(60): n is a, c, g, or u
  misc_feature (64)..(65): n is a, c, g, or u
  misc_feature (79)..(79): n is a, c, g, or u
  misc_feature (81)..(81): n is a, c, g, or u
  misc_feature (86)..(86): n is a, c, g, or u
  misc_feature (91)..(91): n is a, c, g, or u
  misc_feature (97)..(97): n is a, c, g, or u
  misc_feature (101)..(101): n is a, c, g, or u
  misc_feature (109)..(109): n is a, c, g, or u
  misc_feature (111)..(113): n is a, c, g, or u
  misc_feature (115)..(115): n is a, c, g, or u
  misc_feature (118)..(118): n is a, c, g, or u
  misc_feature (136)..(137): n is a, c, g, or u
  misc_feature (139)..(139): n is a, c, g, or u
  misc_feature (164)..(164): n is a, c, g, or u
  misc_feature (189)..(189): n is a, c, g, or u
  misc_feature (191)..(191): n is a, c, g, or u
  misc_feature (193)..(193): n is a, c, g, or u
  misc_feature (202)..(203): n is a, c, g, or u
  misc_feature (209)..(209): n is a, c, g, or u
  misc_feature (212)..(212): n is a, c, g, or u
  misc_feature (227)..(227): n is a, c, g, or u
  misc_feature (229)..(229): n is a, c, g, or u
  misc_feature (234)..(234): n is a, c, g, or u
  misc_feature (244)..(244): n is a, c, g, or u
  misc_feature (251)..(251): n is a, c, g, or u
  misc_feature (253)..(253): n is a, c, g, or u
  misc_feature (256)..(256): n is a, c, g, or u
  misc_feature (262)..(262): n is a, c, g, or u
  misc_feature (265)..(265): n is a, c, g, or u
  misc_feature (269)..(270): n is a, c, g, or u
  misc_feature (275)..(275): n is a, c, g, or u
  misc_feature (283)..(284): n is a, c, g, or u
  misc_feature (286)..(286): n is a, c, g, or u
  misc_feature (290)..(291): n is a, c, g, or u
  misc_feature (312)..(312): n is a, c, g, or u
  misc_feature (322)..(323): n is a, c, g, or u
  misc_feature (325)..(325): n is a, c, g, or u
  misc_feature (341)..(341): n is a, c, g, or u
  misc_feature (347)..(347): n is a, c, g, or u
  misc_feature (350)..(350): n is a, c, g, or u
  misc_feature (359)..(359): n is a, c, g, or u
  misc_feature (362)..(362): n is a, c, g, or u
  misc_feature (374)..(374): n is a, c, g, or u
  misc_feature (377)..(377): n is a, c, g, or u
  misc_feature (387)..(389): n is a, c, g, or u
  misc_feature (392)..(392): n is a, c, g, or u
  misc_feature (394)..(394): n is a, c, g, or u
  misc_feature (415)..(416): n is a, c, g, or u
  misc_feature (419)..(419): n is a, c, g, or u
  misc_feature (428)..(428): n is a, c, g, or u
  misc_feature (431)..(431): n is a, c, g, or u
  misc_feature (434)..(434): n is a, c, g, or u
  misc_feature (442)..(442): n is a, c, g, or u
  misc_feature (444)..(444): n is a, c, g, or u
  misc_feature (446)..(446): n is a, c, g, or u
  misc_feature (448)..(448): n is a, c, g, or u
  misc_feature (457)..(458): n is a, c, g, or u
  misc_feature (460)..(460): n is a, c, g, or u
  misc_feature (476)..(476): n is a, c, g, or u
  misc_feature (479)..(479): n is a, c, g, or u
  misc_feature (481)..(481): n is a, c, g, or u
  misc_feature (491)..(491): n is a, c, g, or u
  misc_feature (496)..(496): n is a, c, g, or u
  misc_feature (499)..(499): n is a, c, g, or u
  misc_feature (507)..(507): n is a, c, g, or u
  misc_feature (554)..(554): n is a, c, g, or u
  misc_feature (556)..(556): n is a, c, g, or u
  misc_feature (559)..(559): n is a, c, g, or u
  misc_feature (565)..(565): n is a, c, g, or u
  misc_feature (571)..(572): n is a, c, g, or u
  misc_feature (574)..(574): n is a, c, g, or u
  misc_feature (578)..(578): n is a, c, g, or u
  misc_feature (585)..(585): n is a, c, g, or u
  misc_feature (587)..(587): n is a, c, g, or u
  misc_feature (601)..(601): n is a, c, g, or u
  misc_feature (607)..(607): n is a, c, g, or u
  misc_feature (611)..(611): n is a, c, g, or u
  misc_feature (619)..(619): n is a, c, g, or u
  misc_feature (623)..(623): n is a, c, g, or u
  misc_feature (626)..(626): n is a, c, g, or u
  misc_feature (628)..(629): n is a, c, g, or u
  misc_feature (634)..(634): n is a, c, g, or u
  misc_feature (639)..(639): n is a, c, g, or u
  misc_feature (641)..(641): n is a, c, g, or u
  misc_feature (655)..(655): n is a, c, g, or u
  misc_feature (664)..(664): n is a, c, g, or u
  misc_feature (667)..(667): n is a, c, g, or u
  misc_feature (673)..(673): n is a, c, g, or u
  misc_feature (682)..(682): n is a, c, g, or u
  misc_feature (691)..(692): n is a, c, g, or u
  misc_feature (694)..(694): n is a, c, g, or u
  misc_feature (696)..(696): n is a, c, g, or u
  misc_feature (700)..(700): n is a, c, g, or u
  misc_feature (703)..(703): n is a, c, g, or u
  misc_feature (708)..(709): n is a, c, g, or u
  misc_feature (711)..(711): n is a, c, g, or u
  misc_feature (713)..(713): n is a, c, g, or u
  misc_feature (716)..(716): n is a, c, g, or u
  misc_feature (718)..(718): n is a, c, g, or u
  misc_feature (721)..(721): n is a, c, g, or u
  misc_feature (730)..(730): n is a, c, g, or u
  misc_feature (733)..(733): n is a, c, g, or u
  misc_feature (758)..(758): n is a, c, g, or u
  misc_feature (761)..(761): n is a, c, g, or u
  misc_feature (764)..(764): n is a, c, g, or u
  misc_feature (768)..(768): n is a, c, g, or u
  misc_feature (799)..(799): n is a, c, g, or u
  misc_feature (801)..(801): n is a, c, g, or u
  misc_feature (819)..(819): n is a, c, g, or u
  misc_feature (830)..(830): n is a, c, g, or u
  misc_feature (834)..(834): n is a, c, g, or u
  misc_feature (836)..(837): n is a, c, g, or u
  misc_feature (839)..(841): n is a, c, g, or u
  misc_feature (843)..(843): n is a, c, g, or u
  misc_feature (845)..(845): n is a, c, g, or u
  misc_feature (861)..(861): n is a, c, g, or u
  misc_feature (864)..(864): n is a, c, g, or u
  misc_feature (874)..(874): n is a, c, g, or u
  misc_feature (880)..(880): n is a, c, g, or u
  misc_feature (882)..(882): n is a, c, g, or u
  misc_feature (886)..(886): n is a, c, g, or u
  misc_feature (891)..(892): n is a, c, g, or u
  misc_feature (894)..(894): n is a, c, g, or u
  misc_feature (897)..(897): n is a, c, g, or u
  misc_feature (915)..(915): n is a, c, g, or u
  misc_feature (918)..(918): n is a, c, g, or u
  misc_feature (929)..(929): n is a, c, g, or u
  misc_feature (932)..(932): n is a, c, g, or u
  misc_feature (935)..(935): n is a, c, g, or u
  misc_feature (943)..(943): n is a, c, g, or u
  misc_feature (950)..(950): n is a, c, g, or u
  misc_feature (952)..(952): n is a, c, g, or u
  misc_feature (960)..(960): n is a, c, g, or u
  misc_feature (970)..(970): n is a, c, g, or u
  misc_feature (981)..(981): n is a, c, g, or u
  misc_feature (985)..(985): n is a, c, g, or u
  misc_feature (990)..(990): n is a, c, g, or u
  misc_feature (1000)..(1000): n is a, c, g, or u
  misc_feature (1002)..(1002): n is a, c, g, or u
  misc_feature (1005)..(1005): n is a, c, g, or u
  misc_feature (1008)..(1008): n is a, c, g, or u
  misc_feature (1019)..(1019): n is a, c, g, or u
  misc_feature (1024)..(1025): n is a, c, g, or u
  misc_feature (1032)..(1032): n is a, c, g, or u
  misc_feature (1034)..(1034): n is a, c, g, or u
  misc_feature (1040)..(1040): n is a, c, g, or u
  misc_feature (1043)..(1043): n is a, c, g, or u
  misc_feature (1052)..(1052): n is a, c, g, or u
  misc_feature (1069)..(1069): n is a, c, g, or u
  misc_feature (1084)..(1084): n is a, c, g, or u
  misc_feature (1087)..(1087): n is a, c, g, or u
  misc_feature (1104)..(1104): n is a, c, g, or u
  misc_feature (1106)..(1106): n is a, c, g, or u
  misc_feature (1127)..(1127): n is a, c, g, or u
  misc_feature (1129)..(1130): n is a, c, g, or u
  misc_feature (1154)..(1154): n is a, c, g, or u
  misc_feature (1165)..(1170): n is a, c, g, or u
  misc_feature (1175)..(1175): n is a, c, g, or u
  misc_feature (1179)..(1179): n is a, c, g, or u
  misc_feature (1187)..(1187): n is a, c, g, or u
  misc_feature (1195)..(1196): n is a, c, g, or u
  misc_feature (1206)..(1206): n is a, c, g, or u
  misc_feature (1223)..(1223): n is a, c, g, or u
  misc_feature (1226)..(1227): n is a, c, g, or u
  misc_feature (1229)..(1229): n is a, c, g, or u
  misc_feature (1232)..(1233): n is a, c, g, or u
  misc_feature (1249)..(1249): n is a, c, g, or u
  misc_feature (1253)..(1253): n is a, c, g, or u
  misc_feature (1256)..(1256): n is a, c, g, or u
  misc_feature (1258)..(1258): n is a, c, g, or u
  misc_feature (1262)..(1262): n is a, c, g, or u
  misc_feature (1283)..(1283): n is a, c, g, or u
  misc_feature (1286)..(1288): n is a, c, g, or u
  misc_feature (1290)..(1290): n is a, c, g, or u
  misc_feature (1300)..(1301): n is a, c, g, or u
  misc_feature (1303)..(1304): n is a, c, g, or u
  misc_feature (1324)..(1325): n is a, c, g, or u
  misc_feature (1337)..(1338): n is a, c, g, or u
  misc_feature (1346)..(1346): n is a, c, g, or u
  misc_feature (1354)..(1354): n is a, c, g, or u
  misc_feature (1356)..(1357): n is a, c, g, or u
  misc_feature (1359)..(1359): n is a, c, g, or u
  misc_feature (1363)..(1363): n is a, c, g, or u
cnggannnnnnncgggnagnggaaaaccagcagccncccgcgacgangccccncaacgnnagcnncaccaacaggaacnangaccncgacnacgacncggngcagccgnannncnacngcgacgaggaggagaacnncnaccagcagcagcagcagagcgagcngcagcccccggcgcccagcgagganancnggaagaaanncgagcngcngcccaccccgccccngnccccnagccgccgcnccgggcncngcncgcccnccnacgnngcggncacacccnncncccnncggggagacaacgacggcggnggcgggagcnncnccacggccgaccagcnggaganggngaccgagcngcngggaggagacanggngaaccagagnnncancngcgacccggacgacgagaccnncancaaaaacancancanccaggacngnangnggagcggcnncncggccgccgccaagcncgncncagagaagcnggccnccnaccaggcngcgcgcaaagacagcggcagcccgaaccccgcccgcggccacagcgncngcnccaccnccagcnngnaccngcaggancngagcgccgccgccncagagngcancgaccccncggnggncnnccccnacccncncaacgacagcagcncgcccaagnccngcgccncgcaagacnccagcgccnncncnccgnccncgganncncngcncnccncgacggagnccnccccgcagggcagccccgagccccnggngcnccangaggagacaccgcccaccaccagcagcgacncngaggaggaacaagaagangaggaagaaancgangnngnnncngnggaaaagaggcaggcnccnggcaaaaggncagagncnggancaccnncngcnggaggccacagcaaaccnccncacagcccacnggnccncaagaggngccacgncnccacacancagcacaacnacgcagcgccncccnccacncggaaggacnanccngcngccaagagggncaagnnggacagngncagagnccngagacagancagcaacaaccgaaaangcaccagccccaggnccncggacaccgaggagaangncaagaggcgaacacacaacgncnnggagcgccagaggaggaacgagcnaaaacggagcnnnnnngcccngcgngaccagancccggagnnggaaaacaangaaaaggcccccaaggnagnnanccnnaaaaaagccacagcanacanccngnccgnccaagcagaggagcaaaagcncannncngaagaggacnngnngcggaaacgacgagaacagnngaaacacaaacnngaacagcnacggaacncnngngcgnaa

SEQ ID NO: 38 - DNA, 47 bp, Artificial Sequence
  5'UTR
gggaaataagagagaaaagaagagtaagaagaaatataagagccacc